European Patent Application EP 4 613 336 A2, published September 10, 2025. Title: NANOPARTICLE COMPOSITIONS FOR SUSTAINED THERAPY. Applicant: UTI LIMITED PARTNERSHIP. The sequence listing filed with the application follows.

SEQUENCE LISTING (409 sequences)

SEQ ID NO: 1 - DNA, 3171 bp, synthetic construct
  misc_feature 1..3171: note = source = /note="Description of Artificial Sequence: Synthetic polynucleotide"
  source 1..3171: mol_type = other DNA
atgggttctctgcaaccgctggccaccttgtacctgctgggtatgctggtcgctagcagcctcggacagcacctgcagaaggactacagagcctactacaccttcggaggtggaggcggctcaggaggtggaagcggcggctctggggacacccgaccacgtttcttggagtactctacgtctgagtgtcatttcttcaatgggacggagcgggtgcggtacctggacagatacttccataaccaggaggagaacgtgcgcttcgacagcgacgtgggggagttccgggcggtgacggagctggggcggcctgatgccgagtactggaacagccagaaggacctcctggagcagaagcggggccgggtggacaactactgcagacacaactacggggttgtggagagcttcacagtgcagcggcgagtccatcctaaggtgactgtgtatccttcaaagacccagcccctgcagcaccataacctcctggtctgttctgtgagtggtttctatccaggcagcattgaagtcaggtggttccggaatggccaggaagagaagactggggtggtgtccacaggcctgatccacaatggagactggaccttccagaccctggtgatgctggaaacagttcctcggagtggagaggtttacacctgccaagtggagcacccaagcgtgacaagccctctcacagtggaatggagagcacggtctgaatctgcacagagcaagtccggaggcggaggcggacggatcgctcggctagaggaaaaagtgaaaaccttgaaagcgcaaaactccgagctggcgtccacggccaacatgctcagggaacaggtggcacagcttaagcagaaagtcatgaaccacgacaaaactcacacatgcccaccgtgcccagcacctgaactcctggggggaccgtcagtcttcctcttccccccaaaacccaaggacaccctcatgatctcccggacccctgaggtcacatgcgtggtggtggacgtgagccacgaagaccctgaggtcaagttcaactggtacgtggacggcgtggaggtgcataatgccaagacaaagccgcgggaggagcagtacaacagcacgtaccgtgtggtcagcgtcctcaccgtcctgcaccaggactggctgaatggcaaggagtacaagtgcaaagtctccaacaaagccctcccagcccccatcgagaaaaccatctccaaagccaaagggcagccccgagaaccacaggtgtgcaccctgcccccatcccgggatgagctgaccaagaaccaggtcagcctgagctgcgcggtcaaaggcttctatcccagcgacatcgccgtggagtgggagagcaatgggcagccggagaacaactacaagaccacgcctcccgtgctggactccgacggctccttcttcctcgtcagcaagctcaccgtggacaagagcaggtggcagcaggggaacgtcttctcatgctccgtgatgcatgaggctctgcacaaccactacacacagaagagcctctccctgtctcccggcggctccggagccacgaacttctctctgttaaagcaagcaggagacgtggaagaaaaccccggtcccatggctatcatctacctcatcctcctgttcaccgctgtgcggggcatcaaagaagaacatgtgatcatccaggccgagttctatctgaatcctgaccaatcaggcgagtttatgtttgactttgatggtgatgagattttccatgtggatatggcaaagaaggagacggtctggcggcttgaagaatttggacgatttgccagctttgaggctcaaggtgcattggccaacatagctgtggacaaagccaacctggaaatcatgacaaagcgctccaactatactccgatcaccaatgtacctccagaggtaactgtgctcacaaacagccctgtggaactgagagagcccaacgtcctcatctgtttcatagacaagttcaccccaccagtggtcaatgtcacgtggcttcgaaatggaaaacctgtcaccacaggagtgtcagagacagtcttcctgcccagggaagaccaccttttccgcaagttccactatctccccttcctgccctcaactgaggacgtttacgactgcagggtggagcactggggcttggatgagcctcttctcaagcactgggagtttgatgctccaagccctctcccagagactacagagtccggaggcggaggcggactgacagatacactccaagcggagacagatcaacttgaagacgagaagtctgcgttgcagaccgagattgccaatctactgaaagagaaggaaaaactggagtttattttggcagcccacgacaaaactcacacatgcccaccgtgcccagcacctgaactcctggggggaccgtcagtcttcctcttccccccaaaacccaaggacaccctcatgatctcccggacccctgaggtcacatgcgtggtggtggacgtgagccacgaagaccctgaggtcaagttcaactggtacgtggacggcgtggaggtgcataatgccaagacaaagccgcgggaggagcagtacaacagcacgtaccgtgtggtcagcgtcctcaccgtcctgcaccaggactggctgaatggcaaggagtacaagtgcaaagtctccaacaaagccctcccagcccccatcgagaaaaccatctccaaagccaaagggcagccccgagaaccacaggtgtacaccctgcccccatgccgggatgagctgaccaagaaccaggtcagcctgtggtgcctggtcaaaggcttctatcccagcgacatcgccgtggagtgggagagcaatgggcagccggagaacaactacaagaccacgcctcccgtgctggactccgacggctccttcttcctctacagcaagctcaccgtggacaagagcaggtggcagcaggggaacgtcttctcatgctccgtgatgcatgaggctctgcacaaccactacacacagaagagcctctccctgtctccgggcggtagtggtagtggtagtggatctctgggtggtatcttcgaggctatgaagatggagctgcgcgatcaccatcaccatcaccataactggagccaccctcagttcgagaagtgttga

SEQ ID NO: 2 - DNA, 2931 bp, synthetic construct
  misc_feature 1..2931: note = source = /note="Description of Artificial Sequence: Synthetic polynucleotide"
  source 1..2931: mol_type = other DNA
atgggttctctgcaaccgctggccaccttgtacctgctgggtatgctggtcgctagcagcctcggacagcacctgcagaaggactacagagcctactacaccttcggaggtggaggcggctcaggaggtggaagcggcggctctggggacacccgaccacgtttcttggagtactctacgtctgagtgtcatttcttcaatgggacggagcgggtgcggtacctggacagatacttccataaccaggaggagaacgtgcgcttcgacagcgacgtgggggagttccgggcggtgacggagctggggcggcctgatgccgagtactggaacagccagaaggacctcctggagcagaagcggggccgggtggacaactactgcagacacaactacggggttgtggagagcttcacagtgcagcggcgagtccatcctaaggtgactgtgtatccttcaaagacccagcccctgcagcaccataacctcctggtctgttctgtgagtggtttctatccaggcagcattgaagtcaggtggttccggaatggccaggaagagaagactggggtggtgtccacaggcctgatccacaatggagactggaccttccagaccctggtgatgctggaaacagttcctcggagtggagaggtttacacctgccaagtggagcacccaagcgtgacaagccctctcacagtggaatggagagcacggtctgaatctgcacagagcaagtccggaggcggaggcggagacaaaactcacacatgcccaccgtgcccagcacctgaactcctggggggaccgtcagtcttcctcttccccccaaaacccaaggacaccctcatgatctcccggacccctgaggtcacatgcgtggtggtggacgtgagccacgaagaccctgaggtcaagttcaactggtacgtggacggcgtggaggtgcataatgccaagacaaagccgcgggaggagcagtacaacagcacgtaccgtgtggtcagcgtcctcaccgtcctgcaccaggactggctgaatggcaaggagtacaagtgcaaagtctccaacaaagccctcccagcccccatcgagaaaaccatctccaaagccaaagggcagccccgagaaccacaggtgtgcaccctgcccccatcccgggatgagctgaccaagaaccaggtcagcctgagctgcgcggtcaaaggcttctatcccagcgacatcgccgtggagtgggagagcaatgggcagccggagaacaactacaagaccacgcctcccgtgctggactccgacggctccttcttcctcgtcagcaagctcaccgtggacaagagcaggtggcagcaggggaacgtcttctcatgctccgtgatgcatgaggctctgcacaaccactacacacagaagagcctctccctgtctcccggcggctccggagccacgaacttctctctgttaaagcaagcaggagacgtggaagaaaaccccggtcccatggctatcatctacctcatcctcctgttcaccgctgtgcggggcatcaaagaagaacatgtgatcatccaggccgagttctatctgaatcctgaccaatcaggcgagtttatgtttgactttgatggtgatgagattttccatgtggatatggcaaagaaggagacggtctggcggcttgaagaatttggacgatttgccagctttgaggctcaaggtgcattggccaacatagctgtggacaaagccaacctggaaatcatgacaaagcgctccaactatactccgatcaccaatgtacctccagaggtaactgtgctcacaaacagccctgtggaactgagagagcccaacgtcctcatctgtttcatagacaagttcaccccaccagtggtcaatgtcacgtggcttcgaaatggaaaacctgtcaccacaggagtgtcagagacagtcttcctgcccagggaagaccaccttttccgcaagttccactatctccccttcctgccctcaactgaggacgtttacgactgcagggtggagcactggggcttggatgagcctcttctcaagcactgggagtttgatgctccaagccctctcccagagactacagagtccggaggcggaggcggagacaaaactcacacatgcccaccgtgcccagcacctgaactcctggggggaccgtcagtcttcctcttccccccaaaacccaaggacaccctcatgatctcccggacccctgaggtcacatgcgtggtggtggacgtgagccacgaagaccctgaggtcaagttcaactggtacgtggacggcgtggaggtgcataatgccaagacaaagccgcgggaggagcagtacaacagcacgtaccgtgtggtcagcgtcctcaccgtcctgcaccaggactggctgaatggcaaggagtacaagtgcaaagtctccaacaaagccctcccagcccccatcgagaaaaccatctccaaagccaaagggcagccccgagaaccacaggtgtacaccctgcccccatgccgggatgagctgaccaagaaccaggtcagcctgtggtgcctggtcaaaggcttctatcccagcgacatcgccgtggagtgggagagcaatgggcagccggagaacaactacaagaccacgcctcccgtgctggactccgacggctccttcttcctctacagcaagctcaccgtggacaagagcaggtggcagcaggggaacgtcttctcatgctccgtgatgcatgaggctctgcacaaccactacacacagaagagcctctccctgtctccgggcggtagtggtagtggtagtggatctctgggtggtatcttcgaggctatgaagatggagctgcgcgatcaccatcaccatcaccataactggagccaccctcagttcgagaagtgttga

SEQ ID NO: 3 - DNA, 3168 bp, synthetic construct
  misc_feature 1..3168: note = source = /note="Description of Artificial Sequence: Synthetic polynucleotide"
  source 1..3168: mol_type = other DNA
atggctatcatctacctcatcctcctgttcaccgctgtgcggggcagatctgcccaccatcccatctgggcccgaatggacgccggaggtggaggctcactagtgccccgaggctctggaggtggaggctctggagactccgaaaggcatttcgtgcaccagttcaagggcgagtgctacttcaccaacgggacgcagcgcatacggctcgtgaccagatacatctacaaccgggaggagtacctgcgcttcgacagcgacgtgggcgagtaccgcgcggtgaccgagctggggcggcactcagccgagtactacaataagcagtacctggagcgaacgcgggccgagctggacacggcgtgcagacacaactacgaggagacggaggtccccacctccctgcggcggcttgaacagcccaatgtcgccatctccctgtccaggacagaggccctcaaccaccacaacactctggtctgttcggtgacagatttctacccagccaagatcaaagtgcgctggttcaggaatggccaggaggagacagtgggggtctcatccacacagcttattaggaatggggactggaccttccaggtcctggtcatgctggagatgacccctcatcagggagaggtctatacctgccatgtggagcatcccagcctgaagagccccatcactgtggagtggagggcacagtccgagtctgcccggagcaagtccggaggcggaggcggacggatcgctcggctagaggaaaaagtgaaaaccttgaaagcgcaaaactccgagctggcgtccacggccaacatgctcagggaacaggtggcacagcttaagcagaaagtcatgaaccacgacaaaactcacacatgcccaccgtgcccagcacctgaactcctggggggaccgtcagtcttcctcttccccccaaaacccaaggacaccctcatgatctcccggacccctgaggtcacatgcgtggtggtggacgtgagccacgaagaccctgaggtcaagttcaactggtacgtggacggcgtggaggtgcataatgccaagacaaagccgcgggaggagcagtacaacagcacgtaccgtgtggtcagcgtcctcaccgtcctgcaccaggactggctgaatggcaaggagtacaagtgcaaggtctccaacaaagccctcccagcccccatcgagaaaaccatctccaaagccaaagggcagccccgagaaccacaggtgtgcaccctgcccccatcccgggatgagctgaccaagaaccaggtcagcctgagctgcgcggtcaaaggcttctatcccagcgacatcgccgtggagtgggagagcaatgggcagccggagaacaactacaagaccacgcctcccgtgctggactccgacggctccttcttcctcgtcagcaagctcaccgtggacaagagtaggtggcagcaggggaacgtcttctcatgctccgtgatgcatgaggctctgcacaaccactacacacagaagagcctctccctgtctcccggcggctccggagccacgaacttctctctgttaaagcaagcaggagacgtggaagaaaaccccggtcccatggctatcatctacctcatcctcctgttcaccgctgtgcggggcgaagacgacattgaggccgaccacgtaggcttctatggtacaactgtttatcagtctcctggagacattggccagtacacacatgaatttgatggtgatgagttgttctatgtggacttggataagaagaaaactgtctggaggcttcctgagtttggccaattgatactctttgagccccaaggtggactgcaaaacatagctgcagaaaaacacaacttgggaatcttgactaagaggtcaaatttcaccccagctaccaatgaggctcctcaagcgactgtgttccccaagtcccctgtgctgctgggtcagcccaacacccttatctgctttgtggacaacatcttcccacctgtgatcaacatcacatggctcagaaatagcaagtcagtcacagacggcgtttatgagaccagcttcctcgtcaaccgtgaccattccttccacaagctgtcttatctcaccttcatcccttctgatgatgacatttatgactgcaaggtggagcactggggcctggaggagccggttctgaaacactgggaacctgagattccagcccccatgtcagagctgacagagtccggaggcggaggcggactgacagatacactccaagcggagacagatcaacttgaagacgagaagtctgcgttgcagaccgagattgccaatctactgaaagagaaggaaaaactggagtttattttggcagcccacgacaaaactcacacatgcccaccgtgcccagcacctgaactcctggggggaccgtcagtcttcctcttccccccaaaacccaaggacaccctcatgatctcccggacccctgaggtcacatgcgtggtggtggacgtgagccacgaagaccctgaggtcaagttcaactggtacgtggacggcgtggaggtgcataatgccaagacaaagccgcgggaggagcagtacaacagcacgtaccgtgtggtcagcgtcctcaccgtcctgcaccaggactggctgaatggcaaggagtacaagtgcaaggtctccaacaaagccctcccagcccccatcgagaaaaccatctccaaagccaaagggcagccccgagaaccacaggtgtacaccctgcccccatgccgggatgagctgaccaagaaccaggtcagcctgtggtgcctggtcaaaggcttctatcccagcgacatcgccgtggagtgggagagcaatgggcagccggagaacaactacaagaccacgcctcccgtgctggactccgacggctccttcttcctctacagcaagctcaccgtggacaagagtaggtggcagcaggggaacgtcttctcatgctccgtgatgcatgaggctctgcacaaccactacacacagaagagcctctccctgtctccgggcggtagtggtagtggtagtggatctctgggtggtatcttcgaggctatgaagatggagctgcgcgatcaccatcaccatcaccataactggagccaccctcagttcgagaagtgttga

SEQ ID NO: 4 - DNA, 2928 bp, synthetic construct
  misc_feature 1..2928: note = source = /note="Description of Artificial Sequence: Synthetic polynucleotide"
  source 1..2928: mol_type = other DNA
atggctatcatctacctcatcctcctgttcaccgctgtgcggggcagatctgcccaccatcccatctgggcccgaatggacgccggaggtggaggctcactagtgccccgaggctctggaggtggaggctctggagactccgaaaggcatttcgtgcaccagttcaagggcgagtgctacttcaccaacgggacgcagcgcatacggctcgtgaccagatacatctacaaccgggaggagtacctgcgcttcgacagcgacgtgggcgagtaccgcgcggtgaccgagctggggcggcactcagccgagtactacaataagcagtacctggagcgaacgcgggccgagctggacacggcgtgcagacacaactacgaggagacggaggtccccacctccctgcggcggcttgaacagcccaatgtcgccatctccctgtccaggacagaggccctcaaccaccacaacactctggtctgttcggtgacagatttctacccagccaagatcaaagtgcgctggttcaggaatggccaggaggagacagtgggggtctcatccacacagcttattaggaatggggactggaccttccaggtcctggtcatgctggagatgacccctcatcagggagaggtctatacctgccatgtggagcatcccagcctgaagagccccatcactgtggagtggagggcacagtccgagtctgcccggagcaagtccggaggcggaggcggagacaaaactcacacatgcccaccgtgcccagcacctgaactcctggggggaccgtcagtcttcctcttccccccaaaacccaaggacaccctcatgatctcccggacccctgaggtcacatgcgtggtggtggacgtgagccacgaagaccctgaggtcaagttcaactggtacgtggacggcgtggaggtgcataatgccaagacaaagccgcgggaggagcagtacaacagcacgtaccgtgtggtcagcgtcctcaccgtcctgcaccaggactggctgaatggcaaggagtacaagtgcaaggtctccaacaaagccctcccagcccccatcgagaaaaccatctccaaagccaaagggcagccccgagaaccacaggtgtgcaccctgcccccatcccgggatgagctgaccaagaaccaggtcagcctgagctgcgcggtcaaaggcttctatcccagcgacatcgccgtggagtgggagagcaatgggcagccggagaacaactacaagaccacgcctcccgtgctggactccgacggctccttcttcctcgtcagcaagctcaccgtggacaagagtaggtggcagcaggggaacgtcttctcatgctccgtgatgcatgaggctctgcacaaccactacacacagaagagcctctccctgtctcccggcggctccggagccacgaacttctctctgttaaagcaagcaggagacgtggaagaaaaccccggtcccatggctatcatctacctcatcctcctgttcaccgctgtgcggggcgaagacgacattgaggccgaccacgtaggcttctatggtacaactgtttatcagtctcctggagacattggccagtacacacatgaatttgatggtgatgagttgttctatgtggacttggataagaagaaaactgtctggaggcttcctgagtttggccaattgatactctttgagccccaaggtggactgcaaaacatagctgcagaaaaacacaacttgggaatcttgactaagaggtcaaatttcaccccagctaccaatgaggctcctcaagcgactgtgttccccaagtcccctgtgctgctgggtcagcccaacacccttatctgctttgtggacaacatcttcccacctgtgatcaacatcacatggctcagaaatagcaagtcagtcacagacggcgtttatgagaccagcttcctcgtcaaccgtgaccattccttccacaagctgtcttatctcaccttcatcccttctgatgatgacatttatgactgcaaggtggagcactggggcctggaggagccggttctgaaacactgggaacctgagattccagcccccatgtcagagctgacagagtccggaggcggaggcggagacaaaactcacacatgcccaccgtgcccagcacctgaactcctggggggaccgtcagtcttcctcttccccccaaaacccaaggacaccctcatgatctcccggacccctgaggtcacatgcgtggtggtggacgtgagccacgaagaccctgaggtcaagttcaactggtacgtggacggcgtggaggtgcataatgccaagacaaagccgcgggaggagcagtacaacagcacgtaccgtgtggtcagcgtcctcaccgtcctgcaccaggactggctgaatggcaaggagtacaagtgcaaggtctccaacaaagccctcccagcccccatcgagaaaaccatctccaaagccaaagggcagccccgagaaccacaggtgtacaccctgcccccatgccgggatgagctgaccaagaaccaggtcagcctgtggtgcctggtcaaaggcttctatcccagcgacatcgccgtggagtgggagagcaatgggcagccggagaacaactacaagaccacgcctcccgtgctggactccgacggctccttcttcctctacagcaagctcaccgtggacaagagtaggtggcagcaggggaacgtcttctcatgctccgtgatgcatgaggctctgcacaaccactacacacagaagagcctctccctgtctccgggcggtagtggtagtggtagtggatctctgggtggtatcttcgaggctatgaagatggagctgcgcgatcaccatcaccatcaccataactggagccaccctcagttcgagaagtgttga

SEQ ID NO: 5 - DNA, 3168 bp, synthetic construct
  misc_feature 1..3168: note = source = /note="Description of Artificial Sequence: Synthetic polynucleotide"
  source 1..3168: mol_type = other DNA
atgggttctctgcaaccgctggccaccttgtacctgctgggtatgctggtcgctagcagcctcggacagcacctgcagaaggactacagagcctactacaccttcggaggtggaggcggctcaggaggtggaagcggcggctctggggacacccgaccacgtttcttggagtactctacgtctgagtgtcatttcttcaatgggacggagcgggtgcggtacctggacagatacttccataaccaggaggagaacgtgcgcttcgacagcgacgtgggggagttccgggcggtgacggagctggggcggcctgatgccgagtactggaacagccagaaggacctcctggagcagaagcggggccgggtggacaactactgcagacacaactacggggttgtggagagcttcacagtgcagcggcgagtccatcctaaggtgactgtgtatccttcaaagacccagcccctgcagcaccataacctcctggtctgttctgtgagtggtttctatccaggcagcattgaagtcaggtggttccggaatggccaggaagagaagactggggtggtgtccacaggcctgatccacaatggagactggaccttccagaccctggtgatgctggaaacagttcctcggagtggagaggtttacacctgccaagtggagcacccaagcgtgacaagccctctcacagtggaatggagagcacggtctgaatctgcacagagcaagtccggaggcggaggcggacggatcgctcggctagaggaaaaagtgaaaaccttgaaagcgcaaaactccgagctggcgtccacggccaacatgctcagggaacaggtggcacagcttaagcagaaagtcatgaaccacgacaaaactcacacatgcccaccgtgcccagcacctgaactcctggggggaccgtcagtcttcctcttccccccaaaacccaaggacaccctcatgatctcccggacccctgaggtcacatgcgtggtggtggacgtgagccacgaagaccctgaggtcaagttcaactggtacgtggacggcgtggaggtgcataatgccaagacaaagccgcgggaggagcagtacaacagcacgtaccgtgtggtcagcgtcctcaccgtcctgcaccaggactggctgaatggcaaggagtacaagtgcaaagtctccaacaaagccctcccagcccccatcgagaaaaccatctccaaagccaaagggcagccccgagaaccacaggtgtacaccctgcccccatgccgggatgagctgaccaagaaccaggtcagcctgtggtgcctggtcaaaggcttctatcccagcgacatcgccgtggagtgggagagcaatgggcagccggagaacaactacaagaccacgcctcccgtgctggactccgacggctccttcttcctctacagcaagctcaccgtggacaagagcaggtggcagcaggggaacgtcttctcatgctccgtgatgcatgaggctctgcacaaccactacacacagaagagcctctccctgtctccgggcggctccggagccacgaacttctctctgttaaagcaagcaggagacgtggaagaaaaccccggtcccatggctatcatctacctcatcctcctgttcaccgctgtgcggggcatcaaagaagaacatgtgatcatccaggccgagttctatctgaatcctgaccaatcaggcgagtttatgtttgactttgatggtgatgagattttccatgtggatatggcaaagaaggagacggtctggcggcttgaagaatttggacgatttgccagctttgaggctcaaggtgcattggccaacatagctgtggacaaagccaacctggaaatcatgacaaagcgctccaactatactccgatcaccaatgtacctccagaggtaactgtgctcacaaacagccctgtggaactgagagagcccaacgtcctcatctgtttcatagacaagttcaccccaccagtggtcaatgtcacgtggcttcgaaatggaaaacctgtcaccacaggagtgtcagagacagtcttcctgcccagggaagaccaccttttccgcaagttccactatctccccttcctgccctcaactgaggacgtttacgactgcagggtggagcactggggcttggatgagcctcttctcaagcactgggagtttgatgctccaagccctctcccagagactacagagtccggaggcggaggcggactgacagatacactccaagcggagacagatcaacttgaagacgagaagtctgcgttgcagaccgagattgccaatctactgaaagagaaggaaaaactggagtttattttggcagcccacgacaaaactcacacatgcccaccgtgcccagcacctgaactcctggggggaccgtcagtcttcctcttccccccaaaacccaaggacaccctcatgatctcccggacccctgaggtcacatgcgtggtggtggacgtgagccacgaagaccctgaggtcaagttcaactggtacgtggacggcgtggaggtgcataatgccaagacaaagccgcgggaggagcagtacaacagcacgtaccgtgtggtcagcgtcctcaccgtcctgcaccaggactggctgaatggcaaggagtacaagtgcaaagtctccaacaaagccctcccagcccccatcgagaaaaccatctccaaagccaaagggcagccccgagaaccacaggtgtgcaccctgcccccatcccgggatgagctgaccaagaaccaggtcagcctgagctgcgcggtcaaaggcttctatcccagcgacatcgccgtggagtgggagagcaatgggcagccggagaacaactacaagaccacgcctcccgtgctggactccgacggctccttcttcctcgtcagcaagctcaccgtggacaagagcaggtggcagcaggggaacgtcttctcatgctccgtgatgcatgaggctctgcacaaccactacacacagaagagcctctccctgtctcccggcggtagtggtagtggtagtggatctctgggtggtatcttcgaggctatgaagatggagctgcgcgatcaccatcaccatcaccataactggagccaccctcagttcgagaagtgt

SEQ ID NO: 6 - DNA, 2928 bp, synthetic construct
  misc_feature 1..2928: note = source = /note="Description of Artificial Sequence: Synthetic polynucleotide"
  source 1..2928: mol_type = other DNA
atgggttctctgcaaccgctggccaccttgtacctgctgggtatgctggtcgctagcagcctcggacagcacctgcagaaggactacagagcctactacaccttcggaggtggaggcggctcaggaggtggaagcggcggctctggggacacccgaccacgtttcttggagtactctacgtctgagtgtcatttcttcaatgggacggagcgggtgcggtacctggacagatacttccataaccaggaggagaacgtgcgcttcgacagcgacgtgggggagttccgggcggtgacggagctggggcggcctgatgccgagtactggaacagccagaaggacctcctggagcagaagcggggccgggtggacaactactgcagacacaactacggggttgtggagagcttcacagtgcagcggcgagtccatcctaaggtgactgtgtatccttcaaagacccagcccctgcagcaccataacctcctggtctgttctgtgagtggtttctatccaggcagcattgaagtcaggtggttccggaatggccaggaagagaagactggggtggtgtccacaggcctgatccacaatggagactggaccttccagaccctggtgatgctggaaacagttcctcggagtggagaggtttacacctgccaagtggagcacccaagcgtgacaagccctctcacagtggaatggagagcacggtctgaatctgcacagagcaagtccggaggcggaggcggagacaaaactcacacatgcccaccgtgcccagcacctgaactcctggggggaccgtcagtcttcctcttccccccaaaacccaaggacaccctcatgatctcccggacccctgaggtcacatgcgtggtggtggacgtgagccacgaagaccctgaggtcaagttcaactggtacgtggacggcgtggaggtgcataatgccaagacaaagccgcgggaggagcagtacaacagcacgtaccgtgtggtcagcgtcctcaccgtcctgcaccaggactggctgaatggcaaggagtacaagtgcaaagtctccaacaaagccctcccagcccccatcgagaaaaccatctccaaagccaaagggcagccccgagaaccacaggtgtacaccctgcccccatgccgggatgagctgaccaagaaccaggtcagcctgtggtgcctggtcaaaggcttctatcccagcgacatcgccgtggagtgggagagcaatgggcagccggagaacaactacaagaccacgcctcccgtgctggactccgacggctccttcttcctctacagcaagctcaccgtggacaagagcaggtggcagcaggggaacgtcttctcatgctccgtgatgcatgaggctctgcacaaccactacacacagaagagcctctccctgtctccgggcggctccggagccacgaacttctctctgttaaagcaagcaggagacgtggaagaaaaccccggtcccatggctatcatctacctcatcctcctgttcaccgctgtgcggggcatcaaagaagaacatgtgatcatccaggccgagttctatctgaatcctgaccaatcaggcgagtttatgtttgactttgatggtgatgagattttccatgtggatatggcaaagaaggagacggtctggcggcttgaagaatttggacgatttgccagctttgaggctcaaggtgcattggccaacatagctgtggacaaagccaacctggaaatcatgacaaagcgctccaactatactccgatcaccaatgtacctccagaggtaactgtgctcacaaacagccctgtggaactgagagagcccaacgtcctcatctgtttcatagacaagttcaccccaccagtggtcaatgtcacgtggcttcgaaatggaaaacctgtcaccacaggagtgtcagagacagtcttcctgcccagggaagaccaccttttccgcaagttccactatctccccttcctgccctcaactgaggacgtttacgactgcagggtggagcactggggcttggatgagcctcttctcaagcactgggagtttgatgctccaagccctctcccagagactacagagtccggaggcggaggcggagacaaaactcacacatgcccaccgtgcccagcacctgaactcctggggggaccgtcagtcttcctcttccccccaaaacccaaggacaccctcatgatctcccggacccctgaggtcacatgcgtggtggtggacgtgagccacgaagaccctgaggtcaagttcaactggtacgtggacggcgtggaggtgcataatgccaagacaaagccgcgggaggagcagtacaacagcacgtaccgtgtggtcagcgtcctcaccgtcctgcaccaggactggctgaatggcaaggagtacaagtgcaaagtctccaacaaagccctcccagcccccatcgagaaaaccatctccaaagccaaagggcagccccgagaaccacaggtgtgcaccctgcccccatcccgggatgagctgaccaagaaccaggtcagcctgagctgcgcggtcaaaggcttctatcccagcgacatcgccgtggagtgggagagcaatgggcagccggagaacaactacaagaccacgcctcccgtgctggactccgacggctccttcttcctcgtcagcaagctcaccgtggacaagagcaggtggcagcaggggaacgtcttctcatgctccgtgatgcatgaggctctgcacaaccactacacacagaagagcctctccctgtctcccggcggtagtggtagtggtagtggatctctgggtggtatcttcgaggctatgaagatggagctgcgcgatcaccatcaccatcaccataactggagccaccctcagttcgagaagtgt

SEQ ID NO: 7 - DNA, 3165 bp, synthetic construct
  misc_feature 1..3165: note = source = /note="Description of Artificial Sequence: Synthetic polynucleotide"
  source 1..3165: mol_type = other DNA
atggctatcatctacctcatcctcctgttcaccgctgtgcggggcagatctgcccaccatcccatctgggcccgaatggacgccggaggtggaggctcactagtgccccgaggctctggaggtggaggctctggagactccgaaaggcatttcgtgcaccagttcaagggcgagtgctacttcaccaacgggacgcagcgcatacggctcgtgaccagatacatctacaaccgggaggagtacctgcgcttcgacagcgacgtgggcgagtaccgcgcggtgaccgagctggggcggcactcagccgagtactacaataagcagtacctggagcgaacgcgggccgagctggacacggcgtgcagacacaactacgaggagacggaggtccccacctccctgcggcggcttgaacagcccaatgtcgccatctccctgtccaggacagaggccctcaaccaccacaacactctggtctgttcggtgacagatttctacccagccaagatcaaagtgcgctggttcaggaatggccaggaggagacagtgggggtctcatccacacagcttattaggaatggggactggaccttccaggtcctggtcatgctggagatgacccctcatcagggagaggtctatacctgccatgtggagcatcccagcctgaagagccccatcactgtggagtggagggcacagtccgagtctgcccggagcaagtccggaggcggaggcggacggatcgctcggctagaggaaaaagtgaaaaccttgaaagcgcaaaactccgagctggcgtccacggccaacatgctcagggaacaggtggcacagcttaagcagaaagtcatgaaccacgacaaaactcacacatgcccaccgtgcccagcacctgaactcctggggggaccgtcagtcttcctcttccccccaaaacccaaggacaccctcatgatctcccggacccctgaggtcacatgcgtggtggtggacgtgagccacgaagaccctgaggtcaagttcaactggtacgtggacggcgtggaggtgcataatgccaagacaaagccgcgggaggagcagtacaacagcacgtaccgtgtggtcagcgtcctcaccgtcctgcaccaggactggctgaatggcaaggagtacaagtgcaaggtctccaacaaagccctcccagcccccatcgagaaaaccatctccaaagccaaagggcagccccgagaaccacaggtgtacaccctgcccccatgccgggatgagctgaccaagaaccaggtcagcctgtggtgcctggtcaaaggcttctatcccagcgacatcgccgtggagtgggagagcaatgggcagccggagaacaactacaagaccacgcctcccgtgctggactccgacggctccttcttcctctacagcaagctcaccgtggacaagagtaggtggcagcaggggaacgtcttctcatgctccgtgatgcatgaggctctgcacaaccactacacacagaagagcctctccctgtctccgggcggctccggagccacgaacttctctctgttaaagcaagcaggagacgtggaagaaaaccccggtcccatggctatcatctacctcatcctcctgttcaccgctgtgcggggcgaagacgacattgaggccgaccacgtaggcttctatggtacaactgtttatcagtctcctggagacattggccagtacacacatgaatttgatggtgatgagttgttctatgtggacttggataagaagaaaactgtctggaggcttcctgagtttggccaattgatactctttgagccccaaggtggactgcaaaacatagctgcagaaaaacacaacttgggaatcttgactaagaggtcaaatttcaccccagctaccaatgaggctcctcaagcgactgtgttccccaagtcccctgtgctgctgggtcagcccaacacccttatctgctttgtggacaacatcttcccacctgtgatcaacatcacatggctcagaaatagcaagtcagtcacagacggcgtttatgagaccagcttcctcgtcaaccgtgaccattccttccacaagctgtcttatctcaccttcatcccttctgatgatgacatttatgactgcaaggtggagcactggggcctggaggagccggttctgaaacactgggaacctgagattccagcccccatgtcagagctgacagagtccggaggcggaggcggactgacagatacactccaagcggagacagatcaacttgaagacgagaagtctgcgttgcagaccgagattgccaatctactgaaagagaaggaaaaactggagtttattttggcagcccacgacaaaactcacacatgcccaccgtgcccagcacctgaactcctggggggaccgtcagtcttcctcttccccccaaaacccaaggacaccctcatgatctcccggacccctgaggtcacatgcgtggtggtggacgtgagccacgaagaccctgaggtcaagttcaactggtacgtggacggcgtggaggtgcataatgccaagacaaagccgcgggaggagcagtacaacagcacgtaccgtgtggtcagcgtcctcaccgtcctgcaccaggactggctgaatggcaaggagtacaagtgcaaggtctccaacaaagccctcccagcccccatcgagaaaaccatctccaaagccaaagggcagccccgagaaccacaggtgtgcaccctgcccccatcccgggatgagctgaccaagaaccaggtcagcctgagctgcgcggtcaaaggcttctatcccagcgacatcgccgtggagtgggagagcaatgggcagccggagaacaactacaagaccacgcctcccgtgctggactccgacggctccttcttcctcgtcagcaagctcaccgtggacaagagtaggtggcagcaggggaacgtcttctcatgctccgtgatgcatgaggctctgcacaaccactacacacagaagagcctctccctgtctcccggcggtagtggtagtggtagtggatctctgggtggtatcttcgaggctatgaagatggagctgcgcgatcaccatcaccatcaccataactggagccaccctcagttcgagaagtgt

SEQ ID NO: 8 - DNA, 2925 bp, synthetic construct
  misc_feature 1..2925: note = source = /note="Description of Artificial Sequence: Synthetic polynucleotide"
  source 1..2925: mol_type = other DNA
atggctatcatctacctcatcctcctgttcaccgctgtgcggggcagatctgcccaccatcccatctgggcccgaatggacgccggaggtggaggctcactagtgccccgaggctctggaggtggaggctctggagactccgaaaggcatttcgtgcaccagttcaagggcgagtgctacttcaccaacgggacgcagcgcatacggctcgtgaccagatacatctacaaccgggaggagtacctgcgcttcgacagcgacgtgggcgagtaccgcgcggtgaccgagctggggcggcactcagccgagtactacaataagcagtacctggagcgaacgcgggccgagctggacacggcgtgcagacacaactacgaggagacggaggtccccacctccctgcggcggcttgaacagcccaatgtcgccatctccctgtccaggacagaggccctcaaccaccacaacactctggtctgttcggtgacagatttctacccagccaagatcaaagtgcgctggttcaggaatggccaggaggagacagtgggggtctcatccacacagcttattaggaatggggactggaccttccaggtcctggtcatgctggagatgacccctcatcagggagaggtctatacctgccatgtggagcatcccagcctgaagagccccatcactgtggagtggagggcacagtccgagtctgcccggagcaagtccggaggcggaggcggagacaaaactcacacatgcccaccgtgcccagcacctgaactcctggggggaccgtcagtcttcctcttccccccaaaacccaaggacaccctcatgatctcccggacccctgaggtcacatgcgtggtggtggacgtgagccacgaagaccctgaggtcaagttcaactggtacgtggacggcgtggaggtgcataatgccaagacaaagccgcgggaggagcagtacaacagcacgtaccgtgtggtcagcgtcctcaccgtcctgcaccaggactggctgaatggcaaggagtacaagtgcaaggtctccaacaaagccctcccagcccccatcgagaaaaccatctccaaagccaaagggcagccccgagaaccacaggtgtacaccctgcccccatgccgggatgagctgaccaagaaccaggtcagcctgtggtgcctggtcaaaggcttctatcccagcgacatcgccgtggagtgggagagcaatgggcagccggagaacaactacaagaccacgcctcccgtgctggactccgacggctccttcttcctctacagcaagctcaccgtggacaagagtaggtggcagcaggggaacgtcttctcatgctccgtgatgcatgaggctctgcacaaccactacacacagaagagcctctccctgtctccgggcggctccggagccacgaacttctctctgttaaagcaagcaggagacgtggaagaaaaccccggtcccatggctatcatctacctcatcctcctgttcaccgctgtgcggggcgaagacgacattgaggccgaccacgtaggcttctatggtacaactgtttatcagtctcctggagacattggccagtacacacatgaatttgatggtgatgagttgttctatgtggacttggataagaagaaaactgtctggaggcttcctgagtttggccaattgatactctttgagccccaaggtggactgcaaaacatagctgcagaaaaacacaacttgggaatcttgactaagaggtcaaatttcaccccagctaccaatgaggctcctcaagcgactgtgttccccaagtcccctgtgctgctgggtcagcccaacacccttatctgctttgtggacaacatcttcccacctgtgatcaacatcacatggctcagaaatagcaagtcagtcacagacggcgtttatgagaccagcttcctcgtcaaccgtgaccattccttccacaagctgtcttatctcaccttcatcccttctgatgatgacatttatgactgcaaggtggagcactggggcctggaggagccggttctgaaacactgggaacctgagattccagcccccatgtcagagctgacagagtccggaggcggaggcggagacaaaactcacacatgcccaccgtgcccagcacctgaactcctggggggaccgtcagtcttcctcttccccccaaaacccaaggacaccctcatgatctcccggacccctgaggtcacatgcgtggtggtggacgtgagccacgaagaccctgaggtcaagttcaactggtacgtggacggcgtggaggtgcataatgccaagacaaagccgcgggaggagcagtacaacagcacgtaccgtgtggtcagcgtcctcaccgtcctgcaccaggactggctgaatggcaaggagtacaagtgcaaggtctccaacaaagccctcccagcccccatcgagaaaaccatctccaaagccaaagggcagccccgagaaccacaggtgtgcaccctgcccccatcccgggatgagctgaccaagaaccaggtcagcctgagctgcgcggtcaaaggcttctatcccagcgacatcgccgtggagtgggagagcaatgggcagccggagaacaactacaagaccacgcctcccgtgctggactccgacggctccttcttcctcgtcagcaagctcaccgtggacaagagtaggtggcagcaggggaacgtcttctcatgctccgtgatgcatgaggctctgcacaaccactacacacagaagagcctctccctgtctcccggcggtagtggtagtggtagtggatctctgggtggtatcttcgaggctatgaagatggagctgcgcgatcaccatcaccatcaccataactggagccaccctcagttcgagaagtgt

SEQ ID NO: 9 - DNA, 1554 bp, synthetic construct
  misc_feature 1..1554: note = source = /note="Description of Artificial Sequence: Synthetic polynucleotide"
  source 1..1554: mol_type = other DNA
atgggttctctgcaaccgctggccaccttgtacctgctgggtatgctggtcgctagcagcctcggacagcacctgcagaaggactacagagcctactacaccttcggaggtggaggcggctcaggaggtggaagcggcggctctggggacacccgaccacgtttcttggagtactctacgtctgagtgtcatttcttcaatgggacggagcgggtgcggtacctggacagatacttccataaccaggaggagaacgtgcgcttcgacagcgacgtgggggagttccgggcggtgacggagctggggcggcctgatgccgagtactggaacagccagaaggacctcctggagcagaagcggggccgggtggacaactactgcagacacaactacggggttgtggagagcttcacagtgcagcggcgagtccatcctaaggtgactgtgtatccttcaaagacccagcccctgcagcaccataacctcctggtctgttctgtgagtggtttctatccaggcagcattgaagtcaggtggttccggaatggccaggaagagaagactggggtggtgtccacaggcctgatccacaatggagactggaccttccagaccctggtgatgctggaaacagttcctcggagtggagaggtttacacctgccaagtggagcacccaagcgtgacaagccctctcacagtggaatggagagcacggtctgaatctgcacagagcaagtccggaggcggaggcggacggatcgctcggctagaggaaaaagtgaaaaccttgaaagcgcaaaactccgagctggcgtccacggccaacatgctcagggaacaggtggcacagcttaagcagaaagtcatgaaccacgacaaaactcacacatgcccaccgtgcccagcacctgaactcctggggggaccgtcagtcttcctcttccccccaaaacccaaggacaccctcatgatctcccggacccctgaggtcacatgcgtggtggtggacgtgagccacgaagaccctgaggtcaagttcaactggtacgtggacggcgtggaggtgcataatgccaagacaaagccgcgggaggagcagtacaacagcacgtaccgtgtggtcagcgtcctcaccgtcctgcaccaggactggctgaatggcaaggagtacaagtgcaaagtctccaacaaagccctcccagcccccatcgagaaaaccatctccaaagccaaagggcagccccgagaaccacaggtgtgcaccctgcccccatcccgggatgagctgaccaagaaccaggtcagcctgagctgcgcggtcaaaggcttctatcccagcgacatcgccgtggagtgggagagcaatgggcagccggagaacaactacaagaccacgcctcccgtgctggactccgacggctccttcttcctcgtcagcaagctcaccgtggacaagagcaggtggcagcaggggaacgtcttctcatgctccgtgatgcatgaggctctgcacaaccactacacacagaagagcctctccctgtctcccggc

SEQ ID NO: 10 - DNA, 1554 bp, synthetic construct
  misc_feature 1..1554: note = source = /note="Description of Artificial Sequence: Synthetic polynucleotide"
  source 1..1554: mol_type = other DNA
atgggttctctgcaaccgctggccaccttgtacctgctgggtatgctggtcgctagcagcctcggacagcacctgcagaaggactacagagcctactacaccttcggaggtggaggcggctcaggaggtggaagcggcggctctggggacacccgaccacgtttcttggagtactctacgtctgagtgtcatttcttcaatgggacggagcgggtgcggtacctggacagatacttccataaccaggaggagaacgtgcgcttcgacagcgacgtgggggagttccgggcggtgacggagctggggcggcctgatgccgagtactggaacagccagaaggacctcctggagcagaagcggggccgggtggacaactactgcagacacaactacggggttgtggagagcttcacagtgcagcggcgagtccatcctaaggtgactgtgtatccttcaaagacccagcccctgcagcaccataacctcctggtctgttctgtgagtggtttctatccaggcagcattgaagtcaggtggttccggaatggccaggaagagaagactggggtggtgtccacaggcctgatccacaatggagactggaccttccagaccctggtgatgctggaaacagttcctcggagtggagaggtttacacctgccaagtggagcacccaagcgtgacaagccctctcacagtggaatggagagcacggtctgaatctgcacagagcaagtccggaggcggaggcggacggatcgctcggctagaggaaaaagtgaaaaccttgaaagcgcaaaactccgagctggcgtccacggccaacatgctcagggaacaggtggcacagcttaagcagaaagtcatgaaccacgacaaaactcacacatgcccaccgtgcccagcacctgaactcctggggggaccgtcagtcttcctcttccccccaaaacccaaggacaccctcatgatctcccggacccctgaggtcacatgcgtggtggtggacgtgagccacgaagaccctgaggtcaagttcaactggtacgtggacggcgtggaggtgcataatgccaagacaaagccgcgggaggagcagtacaacagcacgtaccgtgtggtcagcgtcctcaccgtcctgcaccaggactggctgaatggcaaggagtacaagtgcaaagtctccaacaaagccctcccagcccccatcgagaaaaccatctccaaagccaaagggcagccccgagaaccacaggtgtacaccctgcccccatgccgggatgagctgaccaagaaccaggtcagcctgtggtgcctggtcaaaggcttctatcccagcgacatcgccgtggagtgggagagcaatgggcagccggagaacaactacaagaccacgcctcccgtgctggactccgacggctccttcttcctctacagcaagctcaccgtggacaagagcaggtggcagcaggggaacgtcttctcatgctccgtgatgcatgaggctctgcacaaccactacacacagaagagcctctccctgtctccgggc

SEQ ID NO: 11 - DNA, 1434 bp, synthetic construct
  misc_feature 1..1434: note = source = /note="Description of Artificial Sequence: Synthetic polynucleotide"
  source 1..1434: mol_type = other DNA
atggctatcatctacctcatcctcctgttcaccgctgtgcggggcatcaaagaagaacatgtgatcatccaggccgagttctatctgaatcctgaccaatcaggcgagtttatgtttgactttgatggtgatgagattttccatgtggatatggcaaagaaggagacggtctggcggcttgaagaatttggacgatttgccagctttgaggctcaaggtgcattggccaacatagctgtggacaaagccaacctggaaatcatgacaaagcgctccaactatactccgatcaccaatgtacctccagaggtaactgtgctcacaaacagccctgtggaactgagagagcccaacgtcctcatctgtttcatagacaagttcaccccaccagtggtcaatgtcacgtggcttcgaaatggaaaacctgtcaccacaggagtgtcagagacagtcttcctgcccagggaagaccaccttttccgcaagttccactatctccccttcctgccctcaactgaggacgtttacgactgcagggtggagcactggggcttggatgagcctcttctcaagcactgggagtttgatgctccaagccctctcccagagactacagagtccggaggcggaggcggactgacagatacactccaagcggagacagatcaacttgaagacgagaagtctgcgttgcagaccgagattgccaatctactgaaagagaaggaaaaactggagtttattttggcagcccacgacaaaactcacacatgcccaccgtgcccagcacctgaactcctggggggaccgtcagtcttcctcttccccccaaaacccaaggacaccctcatgatctcccggacccctgaggtcacatgcgtggtggtggacgtgagccacgaagaccctgaggtcaagttcaactggtacgtggacggcgtggaggtgcataatgccaagacaaagccgcgggaggagcagtacaacagcacgtaccgtgtggtcagcgtcctcaccgtcctgcaccaggactggctgaatggcaaggagtacaagtgcaaagtctccaacaaagccctcccagcccccatcgagaaaaccatctccaaagccaaagggcagccccgagaaccacaggtgtacaccctgcccccatgccgggatgagctgaccaagaaccaggtcagcctgtggtgcctggtcaaaggcttctatcccagcgacatcgccgtggagtgggagagcaatgggcagccggagaacaactacaagaccacgcctcccgtgctggactccgacggctccttcttcctctacagcaagctcaccgtggacaagagcaggtggcagcaggggaacgtcttctcatgctccgtgatgcatgaggctctgcacaaccactacacacagaagagcctctccctgtctccgggc

SEQ ID NO: 12 - DNA, 1434 bp, synthetic construct
  misc_feature 1..1434: note = source = /note="Description of Artificial Sequence: Synthetic polynucleotide"
  source 1..1434: mol_type = other DNA
atggctatcatctacctcatcctcctgttcaccgctgtgcggggcatcaaagaagaacatgtgatcatccaggccgagttctatctgaatcctgaccaatcaggcgagtttatgtttgactttgatggtgatgagattttccatgtggatatggcaaagaaggagacggtctggcggcttgaagaatttggacgatttgccagctttgaggctcaaggtgcattggccaacatagctgtggacaaagccaacctggaaatcatgacaaagcgctccaactatactccgatcaccaatgtacctccagaggtaactgtgctcacaaacagccctgtggaactgagagagcccaacgtcctcatctgtttcatagacaagttcaccccaccagtggtcaatgtcacgtggcttcgaaatggaaaacctgtcaccacaggagtgtcagagacagtcttcctgcccagggaagaccaccttttccgcaagttccactatctccccttcctgccctcaactgaggacgtttacgactgcagggtggagcactggggcttggatgagcctcttctcaagcactgggagtttgatgctccaagccctctcccagagactacagagtccggaggcggaggcggactgacagatacactccaagcggagacagatcaacttgaagacgagaagtctgcgttgcagaccgagattgccaatctactgaaagagaaggaaaaactggagtttattttggcagcccacgacaaaactcacacatgcccaccgtgcccagcacctgaactcctggggggaccgtcagtcttcctcttccccccaaaacccaaggacaccctcatgatctcccggacccctgaggtcacatgcgtggtggtggacgtgagccacgaagaccctgaggtcaagttcaactggtacgtggacggcgtggaggtgcataatgccaagacaaagccgcgggaggagcagtacaacagcacgtaccgtgtggtcagcgtcctcaccgtcctgcaccaggactggctgaatggcaaggagtacaagtgcaaagtctccaacaaagccctcccagcccccatcgagaaaaccatctccaaagccaaagggcagccccgagaaccacaggtgtgcaccctgcccccatcccgggatgagctgaccaagaaccaggtcagcctgagctgcgcggtcaaaggcttctatcccagcgacatcgccgtggagtgggagagcaatgggcagccggagaacaactacaagaccacgcctcccgtgctggactccgacggctccttcttcctcgtcagcaagctcaccgtggacaagagcaggtggcagcaggggaacgtcttctcatgctccgtgatgcatgaggctctgcacaaccactacacacagaagagcctctccctgtctcccggc

SEQ ID NO: 13 - DNA, 1434 bp, synthetic construct
  misc_feature 1..1434: note = source = /note="Description of Artificial Sequence: Synthetic polynucleotide"
  source 1..1434: mol_type = other DNA
atgggttctctgcaaccgctggccaccttgtacctgctgggtatgctggtcgctagcagcctcggacagcacctgcagaaggactacagagcctactacaccttcggaggtggaggcggctcaggaggtggaagcggcggctctggggacacccgaccacgtttcttggagtactctacgtctgagtgtcatttcttcaatgggacggagcgggtgcggtacctggacagatacttccataaccaggaggagaacgtgcgcttcgacagcgacgtgggggagttccgggcggtgacggagctggggcggcctgatgccgagtactggaacagccagaaggacctcctggagcagaagcggggccgggtggacaactactgcagacacaactacggggttgtggagagcttcacagtgcagcggcgagtccatcctaaggtgactgtgtatccttcaaagacccagcccctgcagcaccataacctcctggtctgttctgtgagtggtttctatccaggcagcattgaagtcaggtggttccggaatggccaggaagagaagactggggtggtgtccacaggcctgatccacaatggagactggaccttccagaccctggtgatgctggaaacagttcctcggagtggagaggtttacacctgccaagtggagcacccaagcgtgacaagccctctcacagtggaatggagagcacggtctgaatctgcacagagcaagtccggaggcggaggcggagacaaaactcacacatgcccaccgtgcccagcacctgaactcctggggggaccgtcagtcttcctcttccccccaaaacccaaggacaccctcatgatctcccggacccctgaggtcacatgcgtggtggtggacgtgagccacgaagaccctgaggtcaagttcaactggtacgtggacggcgtggaggtgcataatgccaagacaaagccgcgggaggagcagtacaacagcacgtaccgtgtggtcagcgtcctcaccgtcctgcaccaggactggctgaatggcaaggagtacaagtgcaaagtctccaacaaagccctcccagcccccatcgagaaaaccatctccaaagccaaagggcagccccgagaaccacaggtgtgcaccctgcccccatcccgggatgagctgaccaagaaccaggtcagcctgagctgcgcggtcaaaggcttctatcccagcgacatcgccgtggagtgggagagcaatgggcagccggagaacaactacaagaccacgcctcccgtgctggactccgacggctccttcttcctcgtcagcaagctcaccgtggacaagagcaggtggcagcaggggaacgtcttctcatgctccgtgatgcatgaggctctgcacaaccactacacacagaagagcctctccctgtctcccggc

SEQ ID NO: 14 - DNA, 1434 bp, synthetic construct
  misc_feature 1..1434: note = source = /note="Description of Artificial Sequence: Synthetic polynucleotide"
  source 1..1434: mol_type = other DNA
atgggttctctgcaaccgctggccaccttgtacctgctgggtatgctggtcgctagcagcctcggacagcacctgcagaaggactacagagcctactacaccttcggaggtggaggcggctcaggaggtggaagcggcggctctggggacacccgaccacgtttcttggagtactctacgtctgagtgtcatttcttcaatgggacggagcgggtgcggtacctggacagatacttccataaccaggaggagaacgtgcgcttcgacagcgacgtgggggagttccgggcggtgacggagctggggcggcctgatgccgagtactggaacagccagaaggacctcctggagcagaagcggggccgggtggacaactactgcagacacaactacggggttgtggagagcttcacagtgcagcggcgagtccatcctaaggtgactgtgtatccttcaaagacccagcccctgcagcaccataacctcctggtctgttctgtgagtggtttctatccaggcagcattgaagtcaggtggttccggaatggccaggaagagaagactggggtggtgtccacaggcctgatccacaatggagactggaccttccagaccctggtgatgctggaaacagttcctcggagtggagaggtttacacctgccaagtggagcacccaagcgtgacaagccctctcacagtggaatggagagcacggtctgaatctgcacagagcaagtccggaggcggaggcggagacaaaactcacacatgcccaccgtgcccagcacctgaactcctggggggaccgtcagtcttcctcttccccccaaaacccaaggacaccctcatgatctcccggacccctgaggtcacatgcgtggtggtggacgtgagccacgaagaccctgaggtcaagttcaactggtacgtggacggcgtggaggtgcataatgccaagacaaagccgcgggaggagcagtacaacagcacgtaccgtgtggtcagcgtcctcaccgtcctgcaccaggactggctgaatggcaaggagtacaagtgcaaagtctccaacaaagccctcccagcccccatcgagaaaaccatctccaaagccaaagggcagccccgagaaccacaggtgtacaccctgcccccatgccgggatgagctgaccaagaaccaggtcagcctgtggtgcctggtcaaaggcttctatcccagcgacatcgccgtggagtgggagagcaatgggcagccggagaacaactacaagaccacgcctcccgtgctggactccgacggctccttcttcctctacagcaagctcaccgtggacaagagcaggtggcagcaggggaacgtcttctcatgctccgtgatgcatgaggctctgcacaaccactacacacagaagagcctctccctgtctccgggc

SEQ ID NO: 15 - DNA, 1314 bp, synthetic construct
  misc_feature 1..1314: note = source = /note="Description of Artificial Sequence: Synthetic polynucleotide"
  source 1..1314: mol_type = other DNA
atggctatcatctacctcatcctcctgttcaccgctgtgcggggcatcaaagaagaacatgtgatcatccaggccgagttctatctgaatcctgaccaatcaggcgagtttatgtttgactttgatggtgatgagattttccatgtggatatggcaaagaaggagacggtctggcggcttgaagaatttggacgatttgccagctttgaggctcaaggtgcattggccaacatagctgtggacaaagccaacctggaaatcatgacaaagcgctccaactatactccgatcaccaatgtacctccagaggtaactgtgctcacaaacagccctgtggaactgagagagcccaacgtcctcatctgtttcatagacaagttcaccccaccagtggtcaatgtcacgtggcttcgaaatggaaaacctgtcaccacaggagtgtcagagacagtcttcctgcccagggaagaccaccttttccgcaagttccactatctccccttcctgccctcaactgaggacgtttacgactgcagggtggagcactggggcttggatgagcctcttctcaagcactgggagtttgatgctccaagccctctcccagagactacagagtccggaggcggaggcggagacaaaactcacacatgcccaccgtgcccagcacctgaactcctggggggaccgtcagtcttcctcttccccccaaaacccaaggacaccctcatgatctcccggacccctgaggtcacatgcgtggtggtggacgtgagccacgaagaccctgaggtcaagttcaactggtacgtggacggcgtggaggtgcataatgccaagacaaagccgcgggaggagcagtacaacagcacgtaccgtgtggtcagcgtcctcaccgtcctgcaccaggactggctgaatggcaaggagtacaagtgcaaagtctccaacaaagccctcccagcccccatcgagaaaaccatctccaaagccaaagggcagccccgagaaccacaggtgtacaccctgcccccatgccgggatgagctgaccaagaaccaggtcagcctgtggtgcctggtcaaaggcttctatcccagcgacatcgccgtggagtgggagagcaatgggcagccggagaacaactacaagaccacgcctcccgtgctggactccgacggctccttcttcctctacagcaagctcaccgtggacaagagcaggtggcagcaggggaacgtcttctcatgctccgtgatgcatgaggctctgcacaaccactacacacagaagagcctctccctgtctccgggc

SEQ ID NO: 16 - DNA, 1314 bp, synthetic construct
  misc_feature 1..1314: note = source = /note="Description of Artificial Sequence: Synthetic polynucleotide"
  source 1..1314: mol_type = other DNA
atggctatcatctacctcatcctcctgttcaccgctgtgcggggcatcaaagaagaacatgtgatcatccaggccgagttctatctgaatcctgaccaatcaggcgagtttatgtttgactttgatggtgatgagattttccatgtggatatggcaaagaaggagacggtctggcggcttgaagaatttggacgatttgccagctttgaggctcaaggtgcattggccaacatagctgtggacaaagccaacctggaaatcatgacaaagcgctccaactatactccgatcaccaatgtacctccagaggtaactgtgctcacaaacagccctgtggaactgagagagcccaacgtcctcatctgtttcatagacaagttcaccccaccagtggtcaatgtcacgtggcttcgaaatggaaaacctgtcaccacaggagtgtcagagacagtcttcctgcccagggaagaccaccttttccgcaagttccactatctccccttcctgccctcaactgaggacgtttacgactgcagggtggagcactggggcttggatgagcctcttctcaagcactgggagtttgatgctccaagccctctcccagagactacagagtccggaggcggaggcggagacaaaactcacacatgcccaccgtgcccagcacctgaactcctggggggaccgtcagtcttcctcttccccccaaaacccaaggacaccctcatgatctcccggacccctgaggtcacatgcgtggtggtggacgtgagccacgaagaccctgaggtcaagttcaactggtacgtggacggcgtggaggtgcataatgccaagacaaagccgcgggaggagcagtacaacagcacgtaccgtgtggtcagcgtcctcaccgtcctgcaccaggactggctgaatggcaaggagtacaagtgcaaagtctccaacaaagccctcccagcccccatcgagaaaaccatctccaaagccaaagggcagccccgagaaccacaggtgtgcaccctgcccccatcccgggatgagctgaccaagaaccaggtcagcctgagctgcgcggtcaaaggcttctatcccagcgacatcgccgtggagtgggagagcaatgggcagccggagaacaactacaagaccacgcctcccgtgctggactccgacggctccttcttcctcgtcagcaagctcaccgtggacaagagcaggtggcagcaggggaacgtcttctcatgctccgtgatgcatgaggctctgcacaaccactacacacagaagagcctctccctgtctcccggc

SEQ ID NO: 17 - DNA, 1539 bp, synthetic construct
  misc_feature 1..1539: note = source = /note="Description of Artificial Sequence: Synthetic polynucleotide"
  source 1..1539: mol_type = other DNA
atggctatcatctacctcatcctcctgttcaccgctgtgcggggcagatctgcccaccatcccatctgggcccgaatggacgccggaggtggaggctcactagtgccccgaggctctggaggtggaggctctggagactccgaaaggcatttcgtgcaccagttcaagggcgagtgctacttcaccaacgggacgcagcgcatacggctcgtgaccagatacatctacaaccgggaggagtacctgcgcttcgacagcgacgtgggcgagtaccgcgcggtgaccgagctggggcggcactcagccgagtactacaataagcagtacctggagcgaacgcgggccgagctggacacggcgtgcagacacaactacgaggagacggaggtccccacctccctgcggcggcttgaacagcccaatgtcgccatctccctgtccaggacagaggccctcaaccaccacaacactctggtctgttcggtgacagatttctacccagccaagatcaaagtgcgctggttcaggaatggccaggaggagacagtgggggtctcatccacacagcttattaggaatggggactggaccttccaggtcctggtcatgctggagatgacccctcatcagggagaggtctatacctgccatgtggagcatcccagcctgaagagccccatcactgtggagtggagggcacagtccgagtctgcccggagcaagtccggaggcggaggcggacggatcgctcggctagaggaaaaagtgaaaaccttgaaagcgcaaaactccgagctggcgtccacggccaacatgctcagggaacaggtggcacagcttaagcagaaagtcatgaaccacgacaaaactcacacatgcccaccgtgcccagcacctgaactcctggggggaccgtcagtcttcctcttccccccaaaacccaaggacaccctcatgatctcccggacccctgaggtcacatgcgtggtggtggacgtgagccacgaagaccctgaggtcaagttcaactggtacgtggacggcgtggaggtgcataatgccaagacaaagccgcgggaggagcagtacaacagcacgtaccgtgtggtcagcgtcctcaccgtcctgcaccaggactggctgaatggcaaggagtacaagtgcaaggtctccaacaaagccctcccagcccccatcgagaaaaccatctccaaagccaaagggcagccccgagaaccacaggtgtgcaccctgcccccatcccgggatgagctgaccaagaaccaggtcagcctgagctgcgcggtcaaaggcttctatcccagcgacatcgccgtggagtgggagagcaatgggcagccggagaacaactacaagaccacgcctcccgtgctggactccgacggctccttcttcctcgtcagcaagctcaccgtggacaagagtaggtggcagcaggggaacgtcttctcatgctccgtgatgcatgaggctctgcacaaccactacacacagaagagcctctccctgtctcccggc

SEQ ID NO: 18 - DNA, 1539 bp, synthetic construct
  misc_feature 1..1539: note = source = /note="Description of Artificial Sequence: Synthetic polynucleotide"
  source 1..1539: mol_type = other DNA
atggctatcatctacctcatcctcctgttcaccgctgtgcggggcagatctgcccaccatcccatctgggcccgaatggacgccggaggtggaggctcactagtgccccgaggctctggaggtggaggctctggagactccgaaaggcatttcgtgcaccagttcaagggcgagtgctacttcaccaacgggacgcagcgcatacggctcgtgaccagatacatctacaaccgggaggagtacctgcgcttcgacagcgacgtgggcgagtaccgcgcggtgaccgagctggggcggcactcagccgagtactacaataagcagtacctggagcgaacgcgggccgagctggacacggcgtgcagacacaactacgaggagacggaggtccccacctccctgcggcggcttgaacagcccaatgtcgccatctccctgtccaggacagaggccctcaaccaccacaacactctggtctgttcggtgacagatttctacccagccaagatcaaagtgcgctggttcaggaatggccaggaggagacagtgggggtctcatccacacagcttattaggaatggggactggaccttccaggtcctggtcatgctggagatgacccctcatcagggagaggtctatacctgccatgtggagcatcccagcctgaagagccccatcactgtggagtggagggcacagtccgagtctgcccggagcaagtccggaggcggaggcggacggatcgctcggctagaggaaaaagtgaaaaccttgaaagcgcaaaactccgagctggcgtccacggccaacatgctcagggaacaggtggcacagcttaagcagaaagtcatgaaccacgacaaaactcacacatgcccaccgtgcccagcacctgaactcctggggggaccgtcagtcttcctcttccccccaaaacccaaggacaccctcatgatctcccggacccctgaggtcacatgcgtggtggtggacgtgagccacgaagaccctgaggtcaagttcaactggtacgtggacggcgtggaggtgcataatgccaagacaaagccgcgggaggagcagtacaacagcacgtaccgtgtggtcagcgtcctcaccgtcctgcaccaggactggctgaatggcaaggagtacaagtgcaaggtctccaacaaagccctcccagcccccatcgagaaaaccatctccaaagccaaagggcagccccgagaaccacaggtgtacaccctgcccccatgccgggatgagctgaccaagaaccaggtcagcctgtggtgcctggtcaaaggcttctatcccagcgacatcgccgtggagtgggagagcaatgggcagccggagaacaactacaagaccacgcctcccgtgctggactccgacggctccttcttcctctacagcaagctcaccgtggacaagagtaggtggcagcaggggaacgtcttctcatgctccgtgatgcatgaggctctgcacaaccactacacacagaagagcctctccctgtctccgggc

SEQ ID NO: 19 - DNA, 1446 bp, synthetic construct
  misc_feature 1..1446: note = source = /note="Description of Artificial Sequence: Synthetic polynucleotide"
  source 1..1446: mol_type = other DNA
atggctatcatctacctcatcctcctgttcaccgctgtgcggggcgaagacgacattgaggccgaccacgtaggcttctatggtacaactgtttatcagtctcctggagacattggccagtacacacatgaatttgatggtgatgagttgttctatgtggacttggataagaagaaaactgtctggaggcttcctgagtttggccaattgatactctttgagccccaaggtggactgcaaaacatagctgcagaaaaacacaacttgggaatcttgactaagaggtcaaatttcaccccagctaccaatgaggctcctcaagcgactgtgttccccaagtcccctgtgctgctgggtcagcccaacacccttatctgctttgtggacaacatcttcccacctgtgatcaacatcacatggctcagaaatagcaagtcagtcacagacggcgtttatgagaccagcttcctcgtcaaccgtgaccattccttccacaagctgtcttatctcaccttcatcccttctgatgatgacatttatgactgcaaggtggagcactggggcctggaggagccggttctgaaacactgggaacctgagattccagcccccatgtcagagctgacagagtccggaggcggaggcggactgacagatacactccaagcggagacagatcaacttgaagacgagaagtctgcgttgcagaccgagattgccaatctactgaaagagaaggaaaaactggagtttattttggcagcccacgacaaaactcacacatgcccaccgtgcccagcacctgaactcctggggggaccgtcagtcttcctcttccccccaaaacccaaggacaccctcatgatctcccggacccctgaggtcacatgcgtggtggtggacgtgagccacgaagaccctgaggtcaagttcaactggtacgtggacggcgtggaggtgcataatgccaagacaaagccgcgggaggagcagtacaacagcacgtaccgtgtggtcagcgtcctcaccgtcctgcaccaggactggctgaatggcaaggagtacaagtgcaaggtctccaacaaagccctcccagcccccatcgagaaaaccatctccaaagccaaagggcagccccgagaaccacaggtgtacaccctgcccccatgccgggatgagctgaccaagaaccaggtcagcctgtggtgcctggtcaaaggcttctatcccagcgacatcgccgtggagtgggagagcaatgggcagccggagaacaactacaagaccacgcctcccgtgctggactccgacggctccttcttcctctacagcaagctcaccgtggacaagagtaggtggcagcaggggaacgtcttctcatgctccgtgatgcatgaggctctgcacaaccactacacacagaagagcctctccctgtctccgggc

SEQ ID NO: 20 - DNA, 1446 bp, synthetic construct
  misc_feature 1..1446: note = source = /note="Description of Artificial Sequence: Synthetic polynucleotide"
  source 1..1446: mol_type = other DNA
atggctatcatctacctcatcctcctgttcaccgctgtgcggggcgaagacgacattgaggccgaccacgtaggcttctatggtacaactgtttatcagtctcctggagacattggccagtacacacatgaatttgatggtgatgagttgttctatgtggacttggataagaagaaaactgtctggaggcttcctgagtttggccaattgatactctttgagccccaaggtggactgcaaaacatagctgcagaaaaacacaacttgggaatcttgactaagaggtcaaatttcaccccagctaccaatgaggctcctcaagcgactgtgttccccaagtcccctgtgctgctgggtcagcccaacacccttatctgctttgtggacaacatcttcccacctgtgatcaacatcacatggctcagaaatagcaagtcagtcacagacggcgtttatgagaccagcttcctcgtcaaccgtgaccattccttccacaagctgtcttatctcaccttcatcccttctgatgatgacatttatgactgcaaggtggagcactggggcctggaggagccggttctgaaacactgggaacctgagattccagcccccatgtcagagctgacagagtccggaggcggaggcggactgacagatacactccaagcggagacagatcaacttgaagacgagaagtctgcgttgcagaccgagattgccaatctactgaaagagaaggaaaaactggagtttattttggcagcccacgacaaaactcacacatgcccaccgtgcccagcacctgaactcctggggggaccgtcagtcttcctcttccccccaaaacccaaggacaccctcatgatctcccggacccctgaggtcacatgcgtggtggtggacgtgagccacgaagaccctgaggtcaagttcaactggtacgtggacggcgtggaggtgcataatgccaagacaaagccgcgggaggagcagtacaacagcacgtaccgtgtggtcagcgtcctcaccgtcctgcaccaggactggctgaatggcaaggagtacaagtgcaaggtctccaacaaagccctcccagcccccatcgagaaaaccatctccaaagccaaagggcagccccgagaaccacaggtgtgcaccctgcccccatcccgggatgagctgaccaagaaccaggtcagcctgagctgcgcggtcaaaggcttctatcccagcgacatcgccgtggagtgggagagcaatgggcagccggagaacaactacaagaccacgcctcccgtgctggactccgacggctccttcttcctcgtcagcaagctcaccgtggacaagagtaggtggcagcaggggaacgtcttctcatgctccgtgatgcatgaggctctgcacaaccactacacacagaagagcctctccctgtctcccggc

SEQ ID NO: 21 - DNA, 1419 bp, synthetic construct
  misc_feature 1..1419: note = source = /note="Description of Artificial Sequence: Synthetic polynucleotide"
  source 1..1419: mol_type = other DNA
atggctatcatctacctcatcctcctgttcaccgctgtgcggggcagatctgcccaccatcccatctgggcccgaatggacgccggaggtggaggctcactagtgccccgaggctctggaggtggaggctctggagactccgaaaggcatttcgtgcaccagttcaagggcgagtgctacttcaccaacgggacgcagcgcatacggctcgtgaccagatacatctacaaccgggaggagtacctgcgcttcgacagcgacgtgggcgagtaccgcgcggtgaccgagctggggcggcactcagccgagtactacaataagcagtacctggagcgaacgcgggccgagctggacacggcgtgcagacacaactacgaggagacggaggtccccacctccctgcggcggcttgaacagcccaatgtcgccatctccctgtccaggacagaggccctcaaccaccacaacactctggtctgttcggtgacagatttctacccagccaagatcaaagtgcgctggttcaggaatggccaggaggagacagtgggggtctcatccacacagcttattaggaatggggactggaccttccaggtcctggtcatgctggagatgacccctcatcagggagaggtctatacctgccatgtggagcatcccagcctgaagagccccatcactgtggagtggagggcacagtccgagtctgcccggagcaagtccggaggcggaggcggagacaaaactcacacatgcccaccgtgcccagcacctgaactcctggggggaccgtcagtcttcctcttccccccaaaacccaaggacaccctcatgatctcccggacccctgaggtcacatgcgtggtggtggacgtgagccacgaagaccctgaggtcaagttcaactggtacgtggacggcgtggaggtgcataatgccaagacaaagccgcgggaggagcagtacaacagcacgtaccgtgtggtcagcgtcctcaccgtcctgcaccaggactggctgaatggcaaggagtacaagtgcaaggtctccaacaaagccctcccagcccccatcgagaaaaccatctccaaagccaaagggcagccccgagaaccacaggtgtgcaccctgcccccatcccgggatgagctgaccaagaaccaggtcagcctgagctgcgcggtcaaaggcttctatcccagcgacatcgccgtggagtgggagagcaatgggcagccggagaacaactacaagaccacgcctcccgtgctggactccgacggctccttcttcctcgtcagcaagctcaccgtggacaagagtaggtggcagcaggggaacgtcttctcatgctccgtgatgcatgaggctctgcacaaccactacacacagaagagcctctccctgtctcccggc

SEQ ID NO: 22 - DNA, 1419 bp, synthetic construct
  misc_feature 1..1419: note = source = /note="Description of Artificial Sequence: Synthetic polynucleotide"
  source 1..1419: mol_type = other DNA
atggctatcatctacctcatcctcctgttcaccgctgtgcggggcagatctgcccaccatcccatctgggcccgaatggacgccggaggtggaggctcactagtgccccgaggctctggaggtggaggctctggagactccgaaaggcatttcgtgcaccagttcaagggcgagtgctacttcaccaacgggacgcagcgcatacggctcgtgaccagatacatctacaaccgggaggagtacctgcgcttcgacagcgacgtgggcgagtaccgcgcggtgaccgagctggggcggcactcagccgagtactacaataagcagtacctggagcgaacgcgggccgagctggacacggcgtgcagacacaactacgaggagacggaggtccccacctccctgcggcggcttgaacagcccaatgtcgccatctccctgtccaggacagaggccctcaaccaccacaacactctggtctgttcggtgacagatttctacccagccaagatcaaagtgcgctggttcaggaatggccaggaggagacagtgggggtctcatccacacagcttattaggaatggggactggaccttccaggtcctggtcatgctggagatgacccctcatcagggagaggtctatacctgccatgtggagcatcccagcctgaagagccccatcactgtggagtggagggcacagtccgagtctgcccggagcaagtccggaggcggaggcggagacaaaactcacacatgcccaccgtgcccagcacctgaactcctggggggaccgtcagtcttcctcttccccccaaaacccaaggacaccctcatgatctcccggacccctgaggtcacatgcgtggtggtggacgtgagccacgaagaccctgaggtcaagttcaactggtacgtggacggcgtggaggtgcataatgccaagacaaagccgcgggaggagcagtacaacagcacgtaccgtgtggtcagcgtcctcaccgtcctgcaccaggactggctgaatggcaaggagtacaagtgcaaggtctccaacaaagccctcccagcccccatcgagaaaaccatctccaaagccaaagggcagccccgagaaccacaggtgtacaccctgcccccatgccgggatgagctgaccaagaaccaggtcagcctgtggtgcctggtcaaaggcttctatcccagcgacatcgccgtggagtgggagagcaatgggcagccggagaacaactacaagaccacgcctcccgtgctggactccgacggctccttcttcctctacagcaagctcaccgtggacaagagtaggtggcagcaggggaacgtcttctcatgctccgtgatgcatgaggctctgcacaaccactacacacagaagagcctctccctgtctccgggc

SEQ ID NO: 23 - DNA, 1326 bp, synthetic construct
  misc_feature 1..1326: note = source = /note="Description of Artificial Sequence: Synthetic polynucleotide"
  source 1..1326: mol_type = other DNA
atggctatcatctacctcatcctcctgttcaccgctgtgcggggcgaagacgacattgaggccgaccacgtaggcttctatggtacaactgtttatcagtctcctggagacattggccagtacacacatgaatttgatggtgatgagttgttctatgtggacttggataagaagaaaactgtctggaggcttcctgagtttggccaattgatactctttgagccccaaggtggactgcaaaacatagctgcagaaaaacacaacttgggaatcttgactaagaggtcaaatttcaccccagctaccaatgaggctcctcaagcgactgtgttccccaagtcccctgtgctgctgggtcagcccaacacccttatctgctttgtggacaacatcttcccacctgtgatcaacatcacatggctcagaaatagcaagtcagtcacagacggcgtttatgagaccagcttcctcgtcaaccgtgaccattccttccacaagctgtcttatctcaccttcatcccttctgatgatgacatttatgactgcaaggtggagcactggggcctggaggagccggttctgaaacactgggaacctgagattccagcccccatgtcagagctgacagagtccggaggcggaggcggagacaaaactcacacatgcccaccgtgcccagcacctgaactcctggggggaccgtcagtcttcctcttccccccaaaacccaaggacaccctcatgatctcccggacccctgaggtcacatgcgtggtggtggacgtgagccacgaagaccctgaggtcaagttcaactggtacgtggacggcgtggaggtgcataatgccaagacaaagccgcgggaggagcagtacaacagcacgtaccgtgtggtcagcgtcctcaccgtcctgcaccaggactggctgaatggcaaggagtacaagtgcaaggtctccaacaaagccctcccagcccccatcgagaaaaccatctccaaagccaaagggcagccccgagaaccacaggtgtacaccctgcccccatgccgggatgagctgaccaagaaccaggtcagcctgtggtgcctggtcaaaggcttctatcccagcgacatcgccgtggagtgggagagcaatgggcagccggagaacaactacaagaccacgcctcccgtgctggactccgacggctccttcttcctctacagcaagctcaccgtggacaagagtaggtggcagcaggggaacgtcttctcatgctccgtgatgcatgaggctctgcacaaccactacacacagaagagcctctccctgtctccgggc

SEQ ID NO: 24 - DNA, 1326 bp, synthetic construct
  misc_feature 1..1326: note = source = /note="Description of Artificial Sequence: Synthetic polynucleotide"
  source 1..1326: mol_type = other DNA
atggctatcatctacctcatcctcctgttcaccgctgtgcggggcgaagacgacattgaggccgaccacgtaggcttctatggtacaactgtttatcagtctcctggagacattggccagtacacacatgaatttgatggtgatgagttgttctatgtggacttggataagaagaaaactgtctggaggcttcctgagtttggccaattgatactctttgagccccaaggtggactgcaaaacatagctgcagaaaaacacaacttgggaatcttgactaagaggtcaaatttcaccccagctaccaatgaggctcctcaagcgactgtgttccccaagtcccctgtgctgctgggtcagcccaacacccttatctgctttgtggacaacatcttcccacctgtgatcaacatcacatggctcagaaatagcaagtcagtcacagacggcgtttatgagaccagcttcctcgtcaaccgtgaccattccttccacaagctgtcttatctcaccttcatcccttctgatgatgacatttatgactgcaaggtggagcactggggcctggaggagccggttctgaaacactgggaacctgagattccagcccccatgtcagagctgacagagtccggaggcggaggcggagacaaaactcacacatgcccaccgtgcccagcacctgaactcctggggggaccgtcagtcttcctcttccccccaaaacccaaggacaccctcatgatctcccggacccctgaggtcacatgcgtggtggtggacgtgagccacgaagaccctgaggtcaagttcaactggtacgtggacggcgtggaggtgcataatgccaagacaaagccgcgggaggagcagtacaacagcacgtaccgtgtggtcagcgtcctcaccgtcctgcaccaggactggctgaatggcaaggagtacaagtgcaaggtctccaacaaagccctcccagcccccatcgagaaaaccatctccaaagccaaagggcagccccgagaaccacaggtgtgcaccctgcccccatcccgggatgagctgaccaagaaccaggtcagcctgagctgcgcggtcaaaggcttctatcccagcgacatcgccgtggagtgggagagcaatgggcagccggagaacaactacaagaccacgcctcccgtgctggactccgacggctccttcttcctcgtcagcaagctcaccgtggacaagagtaggtggcagcaggggaacgtcttctcatgctccgtgatgcatgaggctctgcacaaccactacacacagaagagcctctccctgtctcccggc

SEQ ID NO: 25 - DNA, 678 bp, synthetic construct
  misc_feature 1..678: note = source = /note="Description of Artificial Sequence: Synthetic polynucleotide"
  source 1..678: mol_type = other DNA
gacaaaactcacacatgcccaccgtgcccagcacctgaactcctggggggaccgtcagtcttcctcttccccccaaaacccaaggacaccctcatgatctcccggacccctgaggtcacatgcgtggtggtggacgtgagccacgaagaccctgaggtcaagttcaactggtacgtggacggcgtggaggtgcataatgccaagacaaagccgcgggaggagcagtacaacagcacgtaccgtgtggtcagcgtcctcaccgtcctgcaccaggactggctgaatggcaaggagtacaagtgcaaagtctccaacaaagccctcccagcccccatcgagaaaaccatctccaaagccaaagggcagccccgagaaccacaggtgtgcaccctgcccccatcccgggatgagctgaccaagaaccaggtcagcctgagctgcgcggtcaaaggcttctatcccagcgacatcgccgtggagtgggagagcaatgggcagccggagaacaactacaagaccacgcctcccgtgctggactccgacggctccttcttcctcgtcagcaagctcaccgtggacaagagcaggtggcagcaggggaacgtcttctcatgctccgtgatgcatgaggctctgcacaaccactacacacagaagagcctctccctgtctcccggc

SEQ ID NO: 26 - DNA, 678 bp, synthetic construct
  misc_feature 1..678: note = source = /note="Description of Artificial Sequence: Synthetic polynucleotide"
  source 1..678: mol_type = other DNA
gacaaaactcacacatgcccaccgtgcccagcacctgaactcctggggggaccgtcagtcttcctcttccccccaaaacccaaggacaccctcatgatctcccggacccctgaggtcacatgcgtggtggtggacgtgagccacgaagaccctgaggtcaagttcaactggtacgtggacggcgtggaggtgcataatgccaagacaaagccgcgggaggagcagtacaacagcacgtaccgtgtggtcagcgtcctcaccgtcctgcaccaggactggctgaatggcaaggagtacaagtgcaaagtctccaacaaagccctcccagcccccatcgagaaaaccatctccaaagccaaagggcagccccgagaaccacaggtgtacaccctgcccccatgccgggatgagctgaccaagaaccaggtcagcctgtggtgcctggtcaaaggcttctatcccagcgacatcgccgtggagtgggagagcaatgggcagccggagaacaactacaagaccacgcctcccgtgctggactccgacggctccttcttcctctacagcaagctcaccgtggacaagagcaggtggcagcaggggaacgtcttctcatgctccgtgatgcatgaggctctgcacaaccactacacacagaagagcctctccctgtctccgggc

SEQ ID NO: 27 - protein, 1056 aa, synthetic construct
  REGION 1..1056: note = source = /note="Description of Artificial Sequence: Synthetic polypeptide"
MGSLQPLATLYLLGMLVASSLGQHLQKDYRAYYTFGGGGGSGGGSGGSGDTRPRFLEYSTSECHFFNGTERVRYLDRYFHNQEENVRFDSDVGEFRAVTELGRPDAEYWNSQKDLLEQKRGRVDNYCRHNYGVVESFTVQRRVHPKVTVYPSKTQPLQHHNLLVCSVSGFYPGSIEVRWFRNGQEEKTGVVSTGLIHNGDWTFQTLVMLETVPRSGEVYTCQVEHPSVTSPLTVEWRARSESAQSKSGGGGGRIARLEEKVKTLKAQNSELASTANMLREQVAQLKQKVMNHDKTHTCPPCPAPELLGGPSVFLFPPKPKDTLMISRTPEVTCVVVDVSHEDPEVKFNWYVDGVEVHNAKTKPREEQYNSTYRVVSVLTVLHQDWLNGKEYKCKVSNKALPAPIEKTISKAKGQPREPQVCTLPPSRDELTKNQVSLSCAVKGFYPSDIAVEWESNGQPENNYKTTPPVLDSDGSFFLVSKLTVDKSRWQQGNVFSCSVMHEALHNHYTQKSLSLSPGGSGATNFSLLKQAGDVEENPGPMAIIYLILLFTAVRGIKEEHVIIQAEFYLNPDQSGEFMFDFDGDEIFHVDMAKKETVWRLEEFGRFASFEAQGALANIAVDKANLEIMTKRSNYTPITNVPPEVTVLTNSPVELREPNVLICFIDKFTPPVVNVTWLRNGKPVTTGVSETVFLPREDHLFRKFHYLPFLPSTEDVYDCRVEHWGLDEPLLKHWEFDAPSPLPETTESGGGGGLTDTLQAETDQLEDEKSALQTEIANLLKEKEKLEFILAAHDKTHTCPPCPAPELLGGPSVFLFPPKPKDTLMISRTPEVTCVVVDVSHEDPEVKFNWYVDGVEVHNAKTKPREEQYNSTYRVVSVLTVLHQDWLNGKEYKCKVSNKALPAPIEKTISKAKGQPREPQVYTLPPCRDELTKNQVSLWCLVKGFYPSDIAVEWESNGQPENNYKTTPPVLDSDGSFFLYSKLTVDKSRWQQGNVFSCSVMHEALHNHYTQKSLSLSPGGSGSGSGSLGGIFEAMKMELRDHHHHHHNWSHPQFEKC

SEQ ID NO: 28 - protein, 976 aa, synthetic construct
  REGION 1..976: note = source = /note="Description of Artificial Sequence: Synthetic polypeptide"
MGSLQPLATLYLLGMLVASSLGQHLQKDYRAYYTFGGGGGSGGGSGGSGDTRPRFLEYSTSECHFFNGTERVRYLDRYFHNQEENVRFDSDVGEFRAVTELGRPDAEYWNSQKDLLEQKRGRVDNYCRHNYGVVESFTVQRRVHPKVTVYPSKTQPLQHHNLLVCSVSGFYPGSIEVRWFRNGQEEKTGVVSTGLIHNGDWTFQTLVMLETVPRSGEVYTCQVEHPSVTSPLTVEWRARSESAQSKSGGGGGDKTHTCPPCPAPELLGGPSVFLFPPKPKDTLMISRTPEVTCVVVDVSHEDPEVKFNWYVDGVEVHNAKTKPREEQYNSTYRVVSVLTVLHQDWLNGKEYKCKVSNKALPAPIEKTISKAKGQPREPQVCTLPPSRDELTKNQVSLSCAVKGFYPSDIAVEWESNGQPENNYKTTPPVLDSDGSFFLVSKLTVDKSRWQQGNVFSCSVMHEALHNHYTQKSLSLSPGGSGATNFSLLKQAGDVEENPGPMAIIYLILLFTAVRGIKEEHVIIQAEFYLNPDQSGEFMFDFDGDEIFHVDMAKKETVWRLEEFGRFASFEAQGALANIAVDKANLEIMTKRSNYTPITNVPPEVTVLTNSPVELREPNVLICFIDKFTPPVVNVTWLRNGKPVTTGVSETVFLPREDHLFRKFHYLPFLPSTEDVYDCRVEHWGLDEPLLKHWEFDAPSPLPETTESGGGGGDKTHTCPPCPAPELLGGPSVFLFPPKPKDTLMISRTPEVTCVVVDVSHEDPEVKFNWYVDGVEVHNAKTKPREEQYNSTYRVVSVLTVLHQDWLNGKEYKCKVSNKALPAPIEKTISKAKGQPREPQVYTLPPCRDELTKNQVSLWCLVKGFYPSDIAVEWESNGQPENNYKTTPPVLDSDGSFFLYSKLTVDKSRWQQGNVFSCSVMHEALHNHYTQKSLSLSPGGSGSGSGSLGGIFEAMKMELRDHHHHHHNWSHPQFEKC

SEQ ID NO: 29 - protein, 1055 aa, synthetic construct
  REGION 1..1055: note = source = /note="Description of Artificial Sequence: Synthetic polypeptide"
MAIIYLILLFTAVRGRSAHHPIWARMDAGGGGSLVPRGSGGGGSGDSERHFVHQFKGECYFTNGTQRIRLVTRYIYNREEYLRFDSDVGEYRAVTELGRHSAEYYNKQYLERTRAELDTACRHNYEETEVPTSLRRLEQPNVAISLSRTEALNHHNTLVCSVTDFYPAKIKVRWFRNGQEETVGVSSTQLIRNGDWTFQVLVMLEMTPHQGEVYTCHVEHPSLKSPITVEWRAQSESARSKSGGGGGRIARLEEKVKTLKAQNSELASTANMLREQVAQLKQKVMNHDKTHTCPPCPAPELLGGPSVFLFPPKPKDTLMISRTPEVTCVVVDVSHEDPEVKFNWYVDGVEVHNAKTKPREEQYNSTYRVVSVLTVLHQDWLNGKEYKCKVSNKALPAPIEKTISKAKGQPREPQVCTLPPSRDELTKNQVSLSCAVKGFYPSDIAVEWESNGQPENNYKTTPPVLDSDGSFFLVSKLTVDKSRWQQGNVFSCSVMHEALHNHYTQKSLSLSPGGSGATNFSLLKQAGDVEENPGPMAIIYLILLFTAVRGEDDIEADHVGFYGTTVYQSPGDIGQYTHEFDGDELFYVDLDKKKTVWRLPEFGQLILFEPQGGLQNIAAEKHNLGILTKRSNFTPATNEAPQATVFPKSPVLLGQPNTLICFVDNIFPPVINITWLRNSKSVTDGVYETSFLVNRDHSFHKLSYLTFIPSDDDIYDCKVEHWGLEEPVLKHWEPEIPAPMSELTESGGGGGLTDTLQAETDQLEDEKSALQTEIANLLKEKEKLEFILAAHDKTHTCPPCPAPELLGGPSVFLFPPKPKDTLMISRTPEVTCVVVDVSHEDPEVKFNWYVDGVEVHNAKTKPREEQYNSTYRVVSVLTVLHQDWLNGKEYKCKVSNKALPAPIEKTISKAKGQPREPQVYTLPPCRDELTKNQVSLWCLVKGFYPSDIAVEWESNGQPENNYKTTPPVLDSDGSFFLYSKLTVDKSRWQQGNVFSCSVMHEALHNHYTQKSLSLSPGGSGSGSGSLGGIFEAMKMELRDHHHHHHNWSHPQFEKC

SEQ ID NO: 30 - protein, 975 aa, synthetic construct
  REGION 1..975: note = source = /note="Description of Artificial Sequence: Synthetic polypeptide"
MAIIYLILLFTAVRGRSAHHPIWARMDAGGGGSLVPRGSGGGGSGDSERHFVHQFKGECYFTNGTQRIRLVTRYIYNREEYLRFDSDVGEYRAVTELGRHSAEYYNKQYLERTRAELDTACRHNYEETEVPTSLRRLEQPNVAISLSRTEALNHHNTLVCSVTDFYPAKIKVRWFRNGQEETVGVSSTQLIRNGDWTFQVLVMLEMTPHQGEVYTCHVEHPSLKSPITVEWRAQSESARSKSGGGGGDKTHTCPPCPAPELLGGPSVFLFPPKPKDTLMISRTPEVTCVVVDVSHEDPEVKFNWYVDGVEVHNAKTKPREEQYNSTYRVVSVLTVLHQDWLNGKEYKCKVSNKALPAPIEKTISKAKGQPREPQVCTLPPSRDELTKNQVSLSCAVKGFYPSDIAVEWESNGQPENNYKTTPPVLDSDGSFFLVSKLTVDKSRWQQGNVFSCSVMHEALHNHYTQKSLSLSPGGSGATNFSLLKQAGDVEENPGPMAIIYLILLFTAVRGEDDIEADHVGFYGTTVYQSPGDIGQYTHEFDGDELFYVDLDKKKTVWRLPEFGQLILFEPQGGLQNIAAEKHNLGILTKRSNFTPATNEAPQATVFPKSPVLLGQPNTLICFVDNIFPPVINITWLRNSKSVTDGVYETSFLVNRDHSFHKLSYLTFIPSDDDIYDCKVEHWGLEEPVLKHWEPEIPAPMSELTESGGGGGDKTHTCPPCPAPELLGGPSVFLFPPKPKDTLMISRTPEVTCVVVDVSHEDPEVKFNWYVDGVEVHNAKTKPREEQYNSTYRVVSVLTVLHQDWLNGKEYKCKVSNKALPAPIEKTISKAKGQPREPQVYTLPPCRDELTKNQVSLWCLVKGFYPSDIAVEWESNGQPENNYKTTPPVLDSDGSFFLYSKLTVDKSRWQQGNVFSCSVMHEALHNHYTQKSLSLSPGGSGSGSGSLGGIFEAMKMELRDHHHHHHNWSHPQFEKC

SEQ ID NO: 31 - protein, 1056 aa, synthetic construct
  REGION 1..1056: note = source = /note="Description of Artificial Sequence: Synthetic polypeptide"
MGSLQPLATLYLLGMLVASSLGQHLQKDYRAYYTFGGGGGSGGGSGGSGDTRPRFLEYSTSECHFFNGTERVRYLDRYFHNQEENVRFDSDVGEFRAVTELGRPDAEYWNSQKDLLEQKRGRVDNYCRHNYGVVESFTVQRRVHPKVTVYPSKTQPLQHHNLLVCSVSGFYPGSIEVRWFRNGQEEKTGVVSTGLIHNGDWTFQTLVMLETVPRSGEVYTCQVEHPSVTSPLTVEWRARSESAQSKSGGGGGRIARLEEKVKTLKAQNSELASTANMLREQVAQLKQKVMNHDKTHTCPPCPAPELLGGPSVFLFPPKPKDTLMISRTPEVTCVVVDVSHEDPEVKFNWYVDGVEVHNAKTKPREEQYNSTYRVVSVLTVLHQDWLNGKEYKCKVSNKALPAPIEKTISKAKGQPREPQVYTLPPCRDELTKNQVSLWCLVKGFYPSDIAVEWESNGQPENNYKTTPPVLDSDGSFFLYSKLTVDKSRWQQGNVFSCSVMHEALHNHYTQKSLSLSPGGSGATNFSLLKQAGDVEENPGPMAIIYLILLFTAVRGIKEEHVIIQAEFYLNPDQSGEFMFDFDGDEIFHVDMAKKETVWRLEEFGRFASFEAQGALANIAVDKANLEIMTKRSNYTPITNVPPEVTVLTNSPVELREPNVLICFIDKFTPPVVNVTWLRNGKPVTTGVSETVFLPREDHLFRKFHYLPFLPSTEDVYDCRVEHWGLDEPLLKHWEFDAPSPLPETTESGGGGGLTDTLQAETDQLEDEKSALQTEIANLLKEKEKLEFILAAHDKTHTCPPCPAPELLGGPSVFLFPPKPKDTLMISRTPEVTCVVVDVSHEDPEVKFNWYVDGVEVHNAKTKPREEQYNSTYRVVSVLTVLHQDWLNGKEYKCKVSNKALPAPIEKTISKAKGQPREPQVCTLPPSRDELTKNQVSLSCAVKGFYPSDIAVEWESNGQPENNYKTTPPVLDSDGSFFLVSKLTVDKSRWQQGNVFSCSVMHEALHNHYTQKSLSLSPGGSGSGSGSLGGIFEAMKMELRDHHHHHHNWSHPQFEKC

SEQ ID NO: 32 - protein, 976 aa, synthetic construct
  REGION 1..976: note = source = /note="Description of Artificial Sequence: Synthetic polypeptide"
MGSLQPLATLYLLGMLVASSLGQHLQKDYRAYYTFGGGGGSGGGSGGSGDTRPRFLEYSTSECHFFNGTERVRYLDRYFHNQEENVRFDSDVGEFRAVTELGRPDAEYWNSQKDLLEQKRGRVDNYCRHNYGVVESFTVQRRVHPKVTVYPSKTQPLQHHNLLVCSVSGFYPGSIEVRWFRNGQEEKTGVVSTGLIHNGDWTFQTLVMLETVPRSGEVYTCQVEHPSVTSPLTVEWRARSESAQSKSGGGGGDKTHTCPPCPAPELLGGPSVFLFPPKPKDTLMISRTPEVTCVVVDVSHEDPEVKFNWYVDGVEVHNAKTKPREEQYNSTYRVVSVLTVLHQDWLNGKEYKCKVSNKALPAPIEKTISKAKGQPREPQVYTLPPCRDELTKNQVSLWCLVKGFYPSDIAVEWESNGQPENNYKTTPPVLDSDGSFFLYSKLTVDKSRWQQGNVFSCSVMHEALHNHYTQKSLSLSPGGSGATNFSLLKQAGDVEENPGPMAIIYLILLFTAVRGIKEEHVIIQAEFYLNPDQSGEFMFDFDGDEIFHVDMAKKETVWRLEEFGRFASFEAQGALANIAVDKANLEIMTKRSNYTPITNVPPEVTVLTNSPVELREPNVLICFIDKFTPPVVNVTWLRNGKPVTTGVSETVFLPREDHLFRKFHYLPFLPSTEDVYDCRVEHWGLDEPLLKHWEFDAPSPLPETTESGGGGGDKTHTCPPCPAPELLGGPSVFLFPPKPKDTLMISRTPEVTCVVVDVSHEDPEVKFNWYVDGVEVHNAKTKPREEQYNSTYRVVSVLTVLHQDWLNGKEYKCKVSNKALPAPIEKTISKAKGQPREPQVCTLPPSRDELTKNQVSLSCAVKGFYPSDIAVEWESNGQPENNYKTTPPVLDSDGSFFLVSKLTVDKSRWQQGNVFSCSVMHEALHNHYTQKSLSLSPGGSGSGSGSLGGIFEAMKMELRDHHHHHHNWSHPQFEKC

SEQ ID NO: 33 - protein, 1055 aa, synthetic construct
  REGION 1..1055: note = source = /note="Description of Artificial Sequence: Synthetic polypeptide"
MAIIYLILLFTAVRGRSAHHPIWARMDAGGGGSLVPRGSGGGGSGDSERHFVHQFKGECYFTNGTQRIRLVTRYIYNREEYLRFDSDVGEYRAVTELGRHSAEYYNKQYLERTRAELDTACRHNYEETEVPTSLRRLEQPNVAISLSRTEALNHHNTLVCSVTDFYPAKIKVRWFRNGQEETVGVSSTQLIRNGDWTFQVLVMLEMTPHQGEVYTCHVEHPSLKSPITVEWRAQSESARSKSGGGGGRIARLEEKVKTLKAQNSELASTANMLREQVAQLKQKVMNHDKTHTCPPCPAPELLGGPSVFLFPPKPKDTLMISRTPEVTCVVVDVSHEDPEVKFNWYVDGVEVHNAKTKPREEQYNSTYRVVSVLTVLHQDWLNGKEYKCKVSNKALPAPIEKTISKAKGQPREPQVYTLPPCRDELTKNQVSLWCLVKGFYPSDIAVEWESNGQPENNYKTTPPVLDSDGSFFLYSKLTVDKSRWQQGNVFSCSVMHEALHNHYTQKSLSLSPGGSGATNFSLLKQAGDVEENPGPMAIIYLILLFTAVRGEDDIEADHVGFYGTTVYQSPGDIGQYTHEFDGDELFYVDLDKKKTVWRLPEFGQLILFEPQGGLQNIAAEKHNLGILTKRSNFTPATNEAPQATVFPKSPVLLGQPNTLICFVDNIFPPVINITWLRNSKSVTDGVYETSFLVNRDHSFHKLSYLTFIPSDDDIYDCKVEHWGLEEPVLKHWEPEIPAPMSELTESGGGGGLTDTLQAETDQLEDEKSALQTEIANLLKEKEKLEFILAAHDKTHTCPPCPAPELLGGPSVFLFPPKPKDTLMISRTPEVTCVVVDVSHEDPEVKFNWYVDGVEVHNAKTKPREEQYNSTYRVVSVLTVLHQDWLNGKEYKCKVSNKALPAPIEKTISKAKGQPREPQVCTLPPSRDELTKNQVSLSCAVKGFYPSDIAVEWESNGQPENNYKTTPPVLDSDGSFFLVSKLTVDKSRWQQGNVFSCSVMHEALHNHYTQKSLSLSPGGSGSGSGSLGGIFEAMKMELRDHHHHHHNWSHPQFEKC

SEQ ID NO: 34 - protein, 975 aa, synthetic construct
  REGION 1..975: note = source = /note="Description of Artificial Sequence: Synthetic polypeptide"
MAIIYLILLFTAVRGRSAHHPIWARMDAGGGGSLVPRGSGGGGSGDSERHFVHQFKGECYFTNGTQRIRLVTRYIYNREEYLRFDSDVGEYRAVTELGRHSAEYYNKQYLERTRAELDTACRHNYEETEVPTSLRRLEQPNVAISLSRTEALNHHNTLVCSVTDFYPAKIKVRWFRNGQEETVGVSSTQLIRNGDWTFQVLVMLEMTPHQGEVYTCHVEHPSLKSPITVEWRAQSESARSKSGGGGGDKTHTCPPCPAPELLGGPSVFLFPPKPKDTLMISRTPEVTCVVVDVSHEDPEVKFNWYVDGVEVHNAKTKPREEQYNSTYRVVSVLTVLHQDWLNGKEYKCKVSNKALPAPIEKTISKAKGQPREPQVYTLPPCRDELTKNQVSLWCLVKGFYPSDIAVEWESNGQPENNYKTTPPVLDSDGSFFLYSKLTVDKSRWQQGNVFSCSVMHEALHNHYTQKSLSLSPGGSGATNFSLLKQAGDVEENPGPMAIIYLILLFTAVRGEDDIEADHVGFYGTTVYQSPGDIGQYTHEFDGDELFYVDLDKKKTVWRLPEFGQLILFEPQGGLQNIAAEKHNLGILTKRSNFTPATNEAPQATVFPKSPVLLGQPNTLICFVDNIFPPVINITWLRNSKSVTDGVYETSFLVNRDHSFHKLSYLTFIPSDDDIYDCKVEHWGLEEPVLKHWEPEIPAPMSELTESGGGGGDKTHTCPPCPAPELLGGPSVFLFPPKPKDTLMISRTPEVTCVVVDVSHEDPEVKFNWYVDGVEVHNAKTKPREEQYNSTYRVVSVLTVLHQDWLNGKEYKCKVSNKALPAPIEKTISKAKGQPREPQVCTLPPSRDELTKNQVSLSCAVKGFYPSDIAVEWESNGQPENNYKTTPPVLDSDGSFFLVSKLTVDKSRWQQGNVFSCSVMHEALHNHYTQKSLSLSPGGSGSGSGSLGGIFEAMKMELRDHHHHHHNWSHPQFEKC

SEQ ID NO: 35 - protein, 518 aa, synthetic construct
  REGION 1..518: note = source = /note="Description of Artificial Sequence: Synthetic polypeptide"
MGSLQPLATLYLLGMLVASSLGQHLQKDYRAYYTFGGGGGSGGGSGGSGDTRPRFLEYSTSECHFFNGTERVRYLDRYFHNQEENVRFDSDVGEFRAVTELGRPDAEYWNSQKDLLEQKRGRVDNYCRHNYGVVESFTVQRRVHPKVTVYPSKTQPLQHHNLLVCSVSGFYPGSIEVRWFRNGQEEKTGVVSTGLIHNGDWTFQTLVMLETVPRSGEVYTCQVEHPSVTSPLTVEWRARSESAQSKSGGGGGRIARLEEKVKTLKAQNSELASTANMLREQVAQLKQKVMNHDKTHTCPPCPAPELLGGPSVFLFPPKPKDTLMISRTPEVTCVVVDVSHEDPEVKFNWYVDGVEVHNAKTKPREEQYNSTYRVVSVLTVLHQDWLNGKEYKCKVSNKALPAPIEKTISKAKGQPREPQVCTLPPSRDELTKNQVSLSCAVKGFYPSDIAVEWESNGQPENNYKTTPPVLDSDGSFFLVSKLTVDKSRWQQGNVFSCSVMHEALHNHYTQKSLSLSPG

SEQ ID NO: 36 - protein, 518 aa, synthetic construct
  REGION 1..518: note = source = /note="Description of Artificial Sequence: Synthetic polypeptide"
MGSLQPLATLYLLGMLVASSLGQHLQKDYRAYYTFGGGGGSGGGSGGSGDTRPRFLEYSTSECHFFNGTERVRYLDRYFHNQEENVRFDSDVGEFRAVTELGRPDAEYWNSQKDLLEQKRGRVDNYCRHNYGVVESFTVQRRVHPKVTVYPSKTQPLQHHNLLVCSVSGFYPGSIEVRWFRNGQEEKTGVVSTGLIHNGDWTFQTLVMLETVPRSGEVYTCQVEHPSVTSPLTVEWRARSESAQSKSGGGGGRIARLEEKVKTLKAQNSELASTANMLREQVAQLKQKVMNHDKTHTCPPCPAPELLGGPSVFLFPPKPKDTLMISRTPEVTCVVVDVSHEDPEVKFNWYVDGVEVHNAKTKPREEQYNSTYRVVSVLTVLHQDWLNGKEYKCKVSNKALPAPIEKTISKAKGQPREPQVYTLPPCRDELTKNQVSLWCLVKGFYPSDIAVEWESNGQPENNYKTTPPVLDSDGSFFLYSKLTVDKSRWQQGNVFSCSVMHEALHNHYTQKSLSLSPG

SEQ ID NO: 37 - protein, 478 aa, synthetic construct
  REGION 1..478: note = source = /note="Description of Artificial Sequence: Synthetic polypeptide"
MAIIYLILLFTAVRGIKEEHVIIQAEFYLNPDQSGEFMFDFDGDEIFHVDMAKKETVWRLEEFGRFASFEAQGALANIAVDKANLEIMTKRSNYTPITNVPPEVTVLTNSPVELREPNVLICFIDKFTPPVVNVTWLRNGKPVTTGVSETVFLPREDHLFRKFHYLPFLPSTEDVYDCRVEHWGLDEPLLKHWEFDAPSPLPETTESGGGGGLTDTLQAETDQLEDEKSALQTEIANLLKEKEKLEFILAAHDKTHTCPPCPAPELLGGPSVFLFPPKPKDTLMISRTPEVTCVVVDVSHEDPEVKFNWYVDGVEVHNAKTKPREEQYNSTYRVVSVLTVLHQDWLNGKEYKCKVSNKALPAPIEKTISKAKGQPREPQVYTLPPCRDELTKNQVSLWCLVKGFYPSDIAVEWESNGQPENNYKTTPPVLDSDGSFFLYSKLTVDKSRWQQGNVFSCSVMHEALHNHYTQKSLSLSPG

SEQ ID NO: 38 - protein, 478 aa, synthetic construct
  REGION 1..478: note = source = /note="Description of Artificial Sequence: Synthetic polypeptide"
MAIIYLILLFTAVRGIKEEHVIIQAEFYLNPDQSGEFMFDFDGDEIFHVDMAKKETVWRLEEFGRFASFEAQGALANIAVDKANLEIMTKRSNYTPITNVPPEVTVLTNSPVELREPNVLICFIDKFTPPVVNVTWLRNGKPVTTGVSETVFLPREDHLFRKFHYLPFLPSTEDVYDCRVEHWGLDEPLLKHWEFDAPSPLPETTESGGGGGLTDTLQAETDQLEDEKSALQTEIANLLKEKEKLEFILAAHDKTHTCPPCPAPELLGGPSVFLFPPKPKDTLMISRTPEVTCVVVDVSHEDPEVKFNWYVDGVEVHNAKTKPREEQYNSTYRVVSVLTVLHQDWLNGKEYKCKVSNKALPAPIEKTISKAKGQPREPQVCTLPPSRDELTKNQVSLSCAVKGFYPSDIAVEWESNGQPENNYKTTPPVLDSDGSFFLVSKLTVDKSRWQQGNVFSCSVMHEALHNHYTQKSLSLSPG

SEQ ID NO: 39 - protein, 478 aa, synthetic construct
  REGION 1..478: note = source = /note="Description of Artificial Sequence: Synthetic polypeptide"
MGSLQPLATLYLLGMLVASSLGQHLQKDYRAYYTFGGGGGSGGGSGGSGDTRPRFLEYSTSECHFFNGTERVRYLDRYFHNQEENVRFDSDVGEFRAVTELGRPDAEYWNSQKDLLEQKRGRVDNYCRHNYGVVESFTVQRRVHPKVTVYPSKTQPLQHHNLLVCSVSGFYPGSIEVRWFRNGQEEKTGVVSTGLIHNGDWTFQTLVMLETVPRSGEVYTCQVEHPSVTSPLTVEWRARSESAQSKSGGGGGDKTHTCPPCPAPELLGGPSVFLFPPKPKDTLMISRTPEVTCVVVDVSHEDPEVKFNWYVDGVEVHNAKTKPREEQYNSTYRVVSVLTVLHQDWLNGKEYKCKVSNKALPAPIEKTISKAKGQPREPQVCTLPPSRDELTKNQVSLSCAVKGFYPSDIAVEWESNGQPENNYKTTPPVLDSDGSFFLVSKLTVDKSRWQQGNVFSCSVMHEALHNHYTQKSLSLSPG

SEQ ID NO: 40 - protein, 478 aa, synthetic construct
  REGION 1..478: note = source = /note="Description of Artificial Sequence: Synthetic polypeptide"
MGSLQPLATLYLLGMLVASSLGQHLQKDYRAYYTFGGGGGSGGGSGGSGDTRPRFLEYSTSECHFFNGTERVRYLDRYFHNQEENVRFDSDVGEFRAVTELGRPDAEYWNSQKDLLEQKRGRVDNYCRHNYGVVESFTVQRRVHPKVTVYPSKTQPLQHHNLLVCSVSGFYPGSIEVRWFRNGQEEKTGVVSTGLIHNGDWTFQTLVMLETVPRSGEVYTCQVEHPSVTSPLTVEWRARSESAQSKSGGGGGDKTHTCPPCPAPELLGGPSVFLFPPKPKDTLMISRTPEVTCVVVDVSHEDPEVKFNWYVDGVEVHNAKTKPREEQYNSTYRVVSVLTVLHQDWLNGKEYKCKVSNKALPAPIEKTISKAKGQPREPQVYTLPPCRDELTKNQVSLWCLVKGFYPSDIAVEWESNGQPENNYKTTPPVLDSDGSFFLYSKLTVDKSRWQQGNVFSCSVMHEALHNHYTQKSLSLSPG

SEQ ID NO: 41 - protein, 438 aa, synthetic construct
  REGION 1..438: note = source = /note="Description of Artificial Sequence: Synthetic polypeptide"
MAIIYLILLFTAVRGIKEEHVIIQAEFYLNPDQSGEFMFDFDGDEIFHVDMAKKETVWRLEEFGRFASFEAQGALANIAVDKANLEIMTKRSNYTPITNVPPEVTVLTNSPVELREPNVLICFIDKFTPPVVNVTWLRNGKPVTTGVSETVFLPREDHLFRKFHYLPFLPSTEDVYDCRVEHWGLDEPLLKHWEFDAPSPLPETTESGGGGGDKTHTCPPCPAPELLGGPSVFLFPPKPKDTLMISRTPEVTCVVVDVSHEDPEVKFNWYVDGVEVHNAKTKPREEQYNSTYRVVSVLTVLHQDWLNGKEYKCKVSNKALPAPIEKTISKAKGQPREPQVYTLPPCRDELTKNQVSLWCLVKGFYPSDIAVEWESNGQPENNYKTTPPVLDSDGSFFLYSKLTVDKSRWQQGNVFSCSVMHEALHNHYTQKSLSLSPG

SEQ ID NO: 42 - protein, 438 aa, synthetic construct
  REGION 1..438: note = source = /note="Description of Artificial Sequence: Synthetic polypeptide"
MAIIYLILLFTAVRGIKEEHVIIQAEFYLNPDQSGEFMFDFDGDEIFHVDMAKKETVWRLEEFGRFASFEAQGALANIAVDKANLEIMTKRSNYTPITNVPPEVTVLTNSPVELREPNVLICFIDKFTPPVVNVTWLRNGKPVTTGVSETVFLPREDHLFRKFHYLPFLPSTEDVYDCRVEHWGLDEPLLKHWEFDAPSPLPETTESGGGGGDKTHTCPPCPAPELLGGPSVFLFPPKPKDTLMISRTPEVTCVVVDVSHEDPEVKFNWYVDGVEVHNAKTKPREEQYNSTYRVVSVLTVLHQDWLNGKEYKCKVSNKALPAPIEKTISKAKGQPREPQVCTLPPSRDELTKNQVSLSCAVKGFYPSDIAVEWESNGQPENNYKTTPPVLDSDGSFFLVSKLTVDKSRWQQGNVFSCSVMHEALHNHYTQKSLSLSPG

SEQ ID NO: 43 - protein, 513 aa, synthetic construct
  REGION 1..513: note = source = /note="Description of Artificial Sequence: Synthetic polypeptide"
MAIIYLILLFTAVRGRSAHHPIWARMDAGGGGSLVPRGSGGGGSGDSERHFVHQFKGECYFTNGTQRIRLVTRYIYNREEYLRFDSDVGEYRAVTELGRHSAEYYNKQYLERTRAELDTACRHNYEETEVPTSLRRLEQPNVAISLSRTEALNHHNTLVCSVTDFYPAKIKVRWFRNGQEETVGVSSTQLIRNGDWTFQVLVMLEMTPHQGEVYTCHVEHPSLKSPITVEWRAQSESARSKSGGGGGRIARLEEKVKTLKAQNSELASTANMLREQVAQLKQKVMNHDKTHTCPPCPAPELLGGPSVFLFPPKPKDTLMISRTPEVTCVVVDVSHEDPEVKFNWYVDGVEVHNAKTKPREEQYNSTYRVVSVLTVLHQDWLNGKEYKCKVSNKALPAPIEKTISKAKGQPREPQVCTLPPSRDELTKNQVSLSCAVKGFYPSDIAVEWESNGQPENNYKTTPPVLDSDGSFFLVSKLTVDKSRWQQGNVFSCSVMHEALHNHYTQKSLSLSPG

SEQ ID NO: 44 - protein, 513 aa, synthetic construct
  REGION 1..513: note = source = /note="Description of Artificial Sequence: Synthetic polypeptide"
MAIIYLILLFTAVRGRSAHHPIWARMDAGGGGSLVPRGSGGGGSGDSERHFVHQFKGECYFTNGTQRIRLVTRYIYNREEYLRFDSDVGEYRAVTELGRHSAEYYNKQYLERTRAELDTACRHNYEETEVPTSLRRLEQPNVAISLSRTEALNHHNTLVCSVTDFYPAKIKVRWFRNGQEETVGVSSTQLIRNGDWTFQVLVMLEMTPHQGEVYTCHVEHPSLKSPITVEWRAQSESARSKSGGGGGRIARLEEKVKTLKAQNSELASTANMLREQVAQLKQKVMNHDKTHTCPPCPAPELLGGPSVFLFPPKPKDTLMISRTPEVTCVVVDVSHEDPEVKFNWYVDGVEVHNAKTKPREEQYNSTYRVVSVLTVLHQDWLNGKEYKCKVSNKALPAPIEKTISKAKGQPREPQVYTLPPCRDELTKNQVSLWCLVKGFYPSDIAVEWESNGQPENNYKTTPPVLDSDGSFFLYSKLTVDKSRWQQGNVFSCSVMHEALHNHYTQKSLSLSPG

SEQ ID NO: 45 - protein, 482 aa, synthetic construct
  REGION 1..482: note = source = /note="Description of Artificial Sequence: Synthetic polypeptide"
MAIIYLILLFTAVRGEDDIEADHVGFYGTTVYQSPGDIGQYTHEFDGDELFYVDLDKKKTVWRLPEFGQLILFEPQGGLQNIAAEKHNLGILTKRSNFTPATNEAPQATVFPKSPVLLGQPNTLICFVDNIFPPVINITWLRNSKSVTDGVYETSFLVNRDHSFHKLSYLTFIPSDDDIYDCKVEHWGLEEPVLKHWEPEIPAPMSELTESGGGGGLTDTLQAETDQLEDEKSALQTEIANLLKEKEKLEFILAAHDKTHTCPPCPAPELLGGPSVFLFPPKPKDTLMISRTPEVTCVVVDVSHEDPEVKFNWYVDGVEVHNAKTKPREEQYNSTYRVVSVLTVLHQDWLNGKEYKCKVSNKALPAPIEKTISKAKGQPREPQVYTLPPCRDELTKNQVSLWCLVKGFYPSDIAVEWESNGQPENNYKTTPPVLDSDGSFFLYSKLTVDKSRWQQGNVFSCSVMHEALHNHYTQKSLSLSPG

SEQ ID NO: 46 - protein, 482 aa, synthetic construct
  REGION 1..482: note = source = /note="Description of Artificial Sequence: Synthetic polypeptide"
MAIIYLILLFTAVRGEDDIEADHVGFYGTTVYQSPGDIGQYTHEFDGDELFYVDLDKKKTVWRLPEFGQLILFEPQGGLQNIAAEKHNLGILTKRSNFTPATNEAPQATVFPKSPVLLGQPNTLICFVDNIFPPVINITWLRNSKSVTDGVYETSFLVNRDHSFHKLSYLTFIPSDDDIYDCKVEHWGLEEPVLKHWEPEIPAPMSELTESGGGGGLTDTLQAETDQLEDEKSALQTEIANLLKEKEKLEFILAAHDKTHTCPPCPAPELLGGPSVFLFPPKPKDTLMISRTPEVTCVVVDVSHEDPEVKFNWYVDGVEVHNAKTKPREEQYNSTYRVVSVLTVLHQDWLNGKEYKCKVSNKALPAPIEKTISKAKGQPREPQVCTLPPSRDELTKNQVSLSCAVKGFYPSDIAVEWESNGQPENNYKTTPPVLDSDGSFFLVSKLTVDKSRWQQGNVFSCSVMHEALHNHYTQKSLSLSPG

SEQ ID NO: 47 - protein, 473 aa, synthetic construct
  REGION 1..473: note = source = /note="Description of Artificial Sequence: Synthetic polypeptide"
MAIIYLILLFTAVRGRSAHHPIWARMDAGGGGSLVPRGSGGGGSGDSERHFVHQFKGECYFTNGTQRIRLVTRYIYNREEYLRFDSDVGEYRAVTELGRHSAEYYNKQYLERTRAELDTACRHNYEETEVPTSLRRLEQPNVAISLSRTEALNHHNTLVCSVTDFYPAKIKVRWFRNGQEETVGVSSTQLIRNGDWTFQVLVMLEMTPHQGEVYTCHVEHPSLKSPITVEWRAQSESARSKSGGGGGDKTHTCPPCPAPELLGGPSVFLFPPKPKDTLMISRTPEVTCVVVDVSHEDPEVKFNWYVDGVEVHNAKTKPREEQYNSTYRVVSVLTVLHQDWLNGKEYKCKVSNKALPAPIEKTISKAKGQPREPQVCTLPPSRDELTKNQVSLSCAVKGFYPSDIAVEWESNGQPENNYKTTPPVLDSDGSFFLVSKLTVDKSRWQQGNVFSCSVMHEALHNHYTQKSLSLSPG

SEQ ID NO: 48 - protein, 473 aa, synthetic construct
  REGION 1..473: note = source = /note="Description of Artificial Sequence: Synthetic polypeptide"
MAIIYLILLFTAVRGRSAHHPIWARMDAGGGGSLVPRGSGGGGSGDSERHFVHQFKGECYFTNGTQRIRLVTRYIYNREEYLRFDSDVGEYRAVTELGRHSAEYYNKQYLERTRAELDTACRHNYEETEVPTSLRRLEQPNVAISLSRTEALNHHNTLVCSVTDFYPAKIKVRWFRNGQEETVGVSSTQLIRNGDWTFQVLVMLEMTPHQGEVYTCHVEHPSLKSPITVEWRAQSESARSKSGGGGGDKTHTCPPCPAPELLGGPSVFLFPPKPKDTLMISRTPEVTCVVVDVSHEDPEVKFNWYVDGVEVHNAKTKPREEQYNSTYRVVSVLTVLHQDWLNGKEYKCKVSNKALPAPIEKTISKAKGQPREPQVYTLPPCRDELTKNQVSLWCLVKGFYPSDIAVEWESNGQPENNYKTTPPVLDSDGSFFLYSKLTVDKSRWQQGNVFSCSVMHEALHNHYTQKSLSLSPG

SEQ ID NO: 49 - protein, 442 aa, synthetic construct
  REGION 1..442: note = source = /note="Description of Artificial Sequence: Synthetic polypeptide"
MAIIYLILLFTAVRGEDDIEADHVGFYGTTVYQSPGDIGQYTHEFDGDELFYVDLDKKKTVWRLPEFGQLILFEPQGGLQNIAAEKHNLGILTKRSNFTPATNEAPQATVFPKSPVLLGQPNTLICFVDNIFPPVINITWLRNSKSVTDGVYETSFLVNRDHSFHKLSYLTFIPSDDDIYDCKVEHWGLEEPVLKHWEPEIPAPMSELTESGGGGGDKTHTCPPCPAPELLGGPSVFLFPPKPKDTLMISRTPEVTCVVVDVSHEDPEVKFNWYVDGVEVHNAKTKPREEQYNSTYRVVSVLTVLHQDWLNGKEYKCKVSNKALPAPIEKTISKAKGQPREPQVYTLPPCRDELTKNQVSLWCLVKGFYPSDIAVEWESNGQPENNYKTTPPVLDSDGSFFLYSKLTVDKSRWQQGNVFSCSVMHEALHNHYTQKSLSLSPG

SEQ ID NO: 50 - protein, 442 aa, synthetic construct
  REGION 1..442: note = source = /note="Description of Artificial Sequence: Synthetic polypeptide"
MAIIYLILLFTAVRGEDDIEADHVGFYGTTVYQSPGDIGQYTHEFDGDELFYVDLDKKKTVWRLPEFGQLILFEPQGGLQNIAAEKHNLGILTKRSNFTPATNEAPQATVFPKSPVLLGQPNTLICFVDNIFPPVINITWLRNSKSVTDGVYETSFLVNRDHSFHKLSYLTFIPSDDDIYDCKVEHWGLEEPVLKHWEPEIPAPMSELTESGGGGGDKTHTCPPCPAPELLGGPSVFLFPPKPKDTLMISRTPEVTCVVVDVSHEDPEVKFNWYVDGVEVHNAKTKPREEQYNSTYRVVSVLTVLHQDWLNGKEYKCKVSNKALPAPIEKTISKAKGQPREPQVCTLPPSRDELTKNQVSLSCAVKGFYPSDIAVEWESNGQPENNYKTTPPVLDSDGSFFLVSKLTVDKSRWQQGNVFSCSVMHEALHNHYTQKSLSLSPG

SEQ ID NO: 51 - protein, 226 aa, synthetic construct
  REGION 1..226: note = source = /note="Description of Artificial Sequence: Synthetic polypeptide"
DKTHTCPPCPAPELLGGPSVFLFPPKPKDTLMISRTPEVTCVVVDVSHEDPEVKFNWYVDGVEVHNAKTKPREEQYNSTYRVVSVLTVLHQDWLNGKEYKCKVSNKALPAPIEKTISKAKGQPREPQVCTLPPSRDELTKNQVSLSCAVKGFYPSDIAVEWESNGQPENNYKTTPPVLDSDGSFFLVSKLTVDKSRWQQGNVFSCSVMHEALHNHYTQKSLSLSPG

SEQ ID NO: 52 - protein, 106 aa, Homo sapiens
GQPREPQVCTLPPSRDELTKNQVSLSCAVKGFYPSDIAVEWESNGQPENNYKTTPPVLDSDGSFFLVSKLTVDKSRWQQGNVFSCSVMHEALHNHYTQKSLSLSPG

SEQ ID NO: 53 - protein, 226 aa, synthetic construct
  REGION 1..226: note = source = /note="Description of Artificial Sequence: Synthetic polypeptide"
DKTHTCPPCPAPELLGGPSVFLFPPKPKDTLMISRTPEVTCVVVDVSHEDPEVKFNWYVDGVEVHNAKTKPREEQYNSTYRVVSVLTVLHQDWLNGKEYKCKVSNKALPAPIEKTISKAKGQPREPQVYTLPPCRDELTKNQVSLWCLVKGFYPSDIAVEWESNGQPENNYKTTPPVLDSDGSFFLYSKLTVDKSRWQQGNVFSCSVMHEALHNHYTQKSLSLSPG

SEQ ID NO: 54 - protein, 106 aa, Homo sapiens
GQPREPQVYTLPPCRDELTKNQVSLWCLVKGFYPSDIAVEWESNGQPENNYKTTPPVLDSDGSFFLYSKLTVDKSRWQQGNVFSCSVMHEALHNHYTQKSLSLSPG

SEQ ID NO: 55 - protein, 113 aa, Homo sapiens
PCPAPELLGGPSVFLFPPKPKDTLMISRTPEVTCVVVDVSHEDPEVKFNWYVDGVEVHNAKTKPREEQYNSTYRVVSVLTVLHQDWLNGKEYKCKVSNKALPAPIEKTISKAK

SEQ ID NO: 56 - protein, 224 aa, synthetic construct
  REGION 1..224: note = source = /note="Description of Artificial Sequence: Synthetic polypeptide"
QHLQKDYRAYYTFGGGGGSGGGSGGSGDTRPRFLEYSTSECHFFNGTERVRYLDRYFHNQEENVRFDSDVGEFRAVTELGRPDAEYWNSQKDLLEQKRGRVDNYCRHNYGVVESFTVQRRVHPKVTVYPSKTQPLQHHNLLVCSVSGFYPGSIEVRWFRNGQEEKTGVVSTGLIHNGDWTFQTLVMLETVPRSGEVYTCQVEHPSVTSPLTVEWRARSESAQSK

SEQ ID NO: 57 - protein, 191 aa, Homo sapiens
IKEEHVIIQAEFYLNPDQSGEFMFDFDGDEIFHVDMAKKETVWRLEEFGRFASFEAQGALANIAVDKANLEIMTKRSNYTPITNVPPEVTVLTNSPVELREPNVLICFIDKFTPPVVNVTWLRNGKPVTTGVSETVFLPREDHLFRKFHYLPFLPSTEDVYDCRVEHWGLDEPLLKHWEFDAPSPLPETTE

SEQ ID NO: 58 - protein, 198 aa, Mus musculus
GDSERHFVHQFKGECYFTNGTQRIRLVTRYIYNREEYLRFDSDVGEYRAVTELGRHSAEYYNKQYLERTRAELDTACRHNYEETEVPTSLRRLEQPNVAISLSRTEALNHHNTLVCSVTDFYPAKIKVRWFRNGQEETVGVSSTQLIRNGDWTFQVLVMLEMTPHQGEVYTCHVEHPSLKSPITVEWRAQSESARSKS

SEQ ID NO: 59 - protein, 196 aa, Mus musculus
EDDIEADHVGFYGTTVYQSPGDIGQYTHEFDGDELFYVDLDKKKTVWRLPEFGQLILFEPQGGLQNIAAEKHNLGILTKRSNFTPATNEAPQATVFPKSPVLLGQPNTLICFVDNIFPPVINITWLRNSKSVTDGVYETSFLVNRDHSFHKLSYLTFIPSDDDIYDCKVEHWGLEEPVLKHWEPEIPAPMSELTES

SEQ ID NO: 60 - protein, 476 aa, synthetic construct
  REGION 1..476: note = source = /note="Description of Artificial Sequence: Synthetic polypeptide"
MAIIYLILLFTAVRGIKEEHVIIQAEFYLNPDQSGEFMFDFDGDEIFHVDMAKKETVWRLEEFGRFASFEAQGALANIAVDKANLECMTKRSNYTPITNVPPEVTVLTNSPVELREPNVLICFIDKFTPPVVNVTWLRNGKPVTTGVSETVFLPREDHLFRKFHYLPFLPSTEDVYDCRVEHWGLDEPLLKHWEFDAPSPLPETTESGGGGGDKTHTCPPCPAPELLGGPSVFLFPPKPKDTLMISRTPEVTCVVVDVSHEDPEVKFNWYVDGVEVHNAKTKPREEQYNSTYRVVSVLTVLHQDWLNGKEYKCKVSNKALPAPIEKTISKAKGQPREPQVYTLPPCRDELTKNQVSLWCLVKGFYPSDIAVEWESNGQPENNYKTTPPVLDSDGSFFLYSKLTVDKSRWQQGNVFSCSVMHEALHNHYTQKSLSLSPGGSGSGSGSLGGIFEAMKMELRDHHHHHHNWSHPQFEKC

SEQ ID NO: 61 - protein, 478 aa, synthetic construct
  REGION 1..478: note = source = /note="Description of Artificial Sequence: Synthetic polypeptide"
MGSLQPLATLYLLGMLVASSLGQHLQKDYRAYYTCGGGGGSGGGSGGSGDTRPRFLEYSTSECHFFNGTERVRYLDRYFHNQEENVRFDSDVGEFRAVTELGRPDAEYWNSQKDLLEQKRGRVDNYCRHNYGVVESFTVQRRVHPKVTVYPSKTQPLQHHNLLVCSVSGFYPGSIEVRWFRNGQEEKTGVVSTGLIHNGDWTFQTLVMLETVPRSGEVYTCQVEHPSVTSPLTVEWRARSESAQSKSGGGGGDKTHTCPPCPAPELLGGPSVFLFPPKPKDTLMISRTPEVTCVVVDVSHEDPEVKFNWYVDGVEVHNAKTKPREEQYNSTYRVVSVLTVLHQDWLNGKEYKCKVSNKALPAPIEKTISKAKGQPREPQVCTLPPSRDELTKNQVSLSCAVKGFYPSDIAVEWESNGQPENNYKTTPPVLDSDGSFFLVSKLTVDKSRWQQGNVFSCSVMHEALHNHYTQKSLSLSPG

SEQ ID NO: 62 - protein, 443 aa, synthetic construct
  REGION 1..443: note = source = /note="Description of Artificial Sequence: Synthetic polypeptide"
MMSFVSLLLVGILFHATQAIKEEHVIIQAEFYLNPDQSGEFMFDFDGDEIFHVDMAKKETVWRLEEFGRFASFEAQGALANIAVDKANLEMTKRSNYTPITNVPPEVTVLTNSVELREPNVLICFIDKFTPVVNVTWLRNGKPVTTGVSETVFLPREDHLFRKFHYLPFLPSTEDVYDCRVEHWGLDEPLLKHWEFDAPSPLPETTESGGGGGDKTHTCPCPAPEAAGGPSVFLFPPKPKDTLMISRTPEVTCVVVDVSHEDPEVKFNWYVDGVEVHNAKTKPREEQYNSTYRVVSVLTVLHQDWLNGKEYKCKVSNKALPAPIEKTISKAKGQPREPQVYTLPPCRDELTKNQVSLWCLVKGFYPSDIAVEWESNGQPENNYKTTPPVLDSDGSFFLYSKLTVDKSRWQQGNVFSCSVMHEALHNHYTQKSLSLSPGGSGSC

SEQ ID NO: 63 - protein, 478 aa, synthetic construct
  REGION 1..478: note = source = /note="Description of Artificial Sequence: Synthetic polypeptide"
MGSLQPLATLYLLGMLVASSLGQHLQKDYRAYYTCGGGGGSGGGSGGSGDTRPRFLEYSTSECHFFNGTERVRYLDRYFHNQEENVRFDSDVGEFRAVTELGRPDAEYWNSQKDLLEQKRGRVDNYCRHNYGVVESFTVQRRVHPKVTVYPSKTQPLQHHNLLVCSVSGFYPGSIEVRWFRNGQEEKTGVVSTGLIHNGDWTFQTLVMLETVPRSGEVYTCQVEHPSVTSPLTVEWRARSESAQSKSGGGGGDKTHTCPPCPAPEAAGGPSVFLFPPKPKDTLMISRTPEVTCVVVDVSHEDPEVKFNWYVDGVEVHNAKTKPREEQYNSTYRVVSVLTVLHQDWLNGKEYKCKVSNKALPAPIEKTISKAKGQPREPQVCTLPPSRDELTKNQVSLSCAVKGFYPSDIAVEWESNGQPENNYKTTPPVLDSDGSFFLVSKLTVDKSRWQQGNVFSCSVMHEALHNHYTQKSLSLSPG

SEQ ID NO: 64 - DNA, 1344 bp, synthetic construct
  misc_feature 1..1344: note = source = /note="Description of Artificial Sequence: Synthetic polynucleotide"
  source 1..1344: mol_type = other DNA
atgatgagcttcgtgagcctgctgctggtgggcatcctgttccacgccacccaggccatcaaagaagaacatgtgatcatccaggccgagttctatctgaatcctgaccaatcaggcgagtttatgtttgactttgatggtgatgagattttccatgtggatatggcaaagaaggagacggtctggcggcttgaagaatttggacgatttgccagctttgaggctcaaggtgcattggccaacatagctgtggacaaagccaacctggaatgcatgacaaagcgctccaactatactccgatcaccaatgtacctccagaggtaactgtgctcacaaacagccctgtggaactgagagagcccaacgtcctcatctgtttcatagacaagttcaccccaccagtggtcaatgtcacgtggcttcgaaatggaaaacctgtcaccacaggagtgtcagagacagtcttcctgcccagggaagaccaccttttccgcaagttccactatctccccttcctgccctcaactgaggacgtttacgactgcagggtggagcactggggcttggatgagcctcttctcaagcactgggagtttgatgctccaagccctctcccagagactacagagtccggaggcggaggcggagacaaaactcacacatgcccaccgtgcccagcacctgaagccgcggggggaccgtcagtcttcctcttccccccaaaacccaaggacaccctcatgatctcccggacccctgaggtcacatgcgtggtggtggacgtgagccacgaagaccctgaggtcaagttcaactggtacgtggacggcgtggaggtgcataatgccaagacaaagccgcgggaggagcagtacaacagcacgtaccgtgtggtcagcgtcctcaccgtcctgcaccaggactggctgaatggcaaggagtacaagtgcaaggtctccaacaaagccctcccagcccccatcgagaaaaccatctccaaagccaaagggcagccccgagaaccacaggtgtacaccctgcccccatgccgggatgagctgaccaagaaccaggtcagcctgtggtgcctggtcaaaggcttctatcccagcgacatcgccgtggagtgggagagcaatgggcagccggagaacaactacaagaccacgcctcccgtgctggactccgacggctccttcttcctctacagcaagctcaccgtggacaagagtaggtggcagcaggggaacgtcttctcatgctccgtgatgcatgaggctctgcacaaccactacacacagaagagcctctccctgtctccgggcggtagtggtagttgttga

SEQ ID NO: 65 - DNA, 1437 bp, synthetic construct
  misc_feature 1..1437: note = source = /note="Description of Artificial Sequence: Synthetic polynucleotide"
  source 1..1437: mol_type = other DNA
atgggttctctgcaaccgctggccaccttgtacctgctgggtatgctggtcgctagcagcctcggacagcacctgcagaaggactacagagcctactacacctgtggaggtggaggcggctcaggaggtggaagcggcggctctggggacacccgaccacgtttcttggagtactctacgtctgagtgtcatttcttcaatgggacggagcgggtgcggtacctggacagatacttccataaccaggaggagaacgtgcgcttcgacagcgacgtgggggagttccgggcggtgacggagctggggcggcctgatgccgagtactggaacagccagaaggacctcctggagcagaagcggggccgggtggacaactactgcagacacaactacggggttgtggagagcttcacagtgcagcggcgagtccatcctaaggtgactgtgtatccttcaaagacccagcccctgcagcaccataacctcctggtctgttctgtgagtggtttctatccaggcagcattgaagtcaggtggttccggaatggccaggaagagaagactggggtggtgtccacaggcctgatccacaatggagactggaccttccagaccctggtgatgctggaaacagttcctcggagtggagaggtttacacctgccaagtggagcacccaagcgtgacaagccctctcacagtggaatggagagcacggtctgaatctgcacagagcaagtccggaggcggaggcggagacaaaactcacacatgcccaccgtgcccagcacctgaagccgcggggggaccgtcagtcttcctcttccccccaaaacccaaggacaccctcatgatctcccggacccctgaggtcacatgcgtggtggtggacgtgagccacgaagaccctgaggtcaagttcaactggtacgtggacggcgtggaggtgcataatgccaagacaaagccgcgggaggagcagtacaacagcacgtaccgtgtggtcagcgtcctcaccgtcctgcaccaggactggctgaatggcaaggagtacaagtgcaaagtctccaacaaagccctcccagcccccatcgagaaaaccatctccaaagccaaagggcagccccgagaaccacaggtgtgcaccctgcccccatcccgggatgagctgaccaagaaccaggtcagcctgagctgcgcggtcaaaggcttctatcccagcgacatcgccgtggagtgggagagcaatgggcagccggagaacaactacaagaccacgcctcccgtgctggactccgacggctccttcttcctcgtcagcaagctcaccgtggacaagagcaggtggcagcaggggaacgtcttctcatgctccgtgatgcatgaggctctgcacaaccactacacacagaagagcctctccctgtctcccggctga

SEQ ID NO: 66 - protein, 9 aa, unidentified
  REGION 1..9: note = source = /note="Description of Unknown: hInsB10-18 sequence"
HLVEALYLV

SEQ ID NO: 67 - protein, 9 aa, unidentified
  REGION 1..9: note = source = /note="Description of Unknown: hIGRP228-236 sequence"
LNIDLLWSV

SEQ ID NO: 68 - protein, 9 aa, unidentified
  REGION 1..9: note = source = /note="Description of Unknown: hIGRP265-273 sequence"
VLFGLGFAI

SEQ ID NO: 69 - protein, 9 aa, unidentified
  REGION 1..9: note = source = /note="Description of Unknown: IGRP206-214 sequence"
VYLKTNVFL

SEQ ID NO: 70 - protein, 9 aa, unidentified
  REGION 1..9: note = source = /note="Description of Unknown: hIGRP206-214 sequence"
VYLKTNLFL

SEQ ID NO: 71 - protein, 9 aa, unidentified
  REGION 1..9: note = source = /note="Description of Unknown: NRP-A7 sequence"
KYNKANAFL

SEQ ID NO: 72 - protein, 9 aa, unidentified
  REGION 1..9: note = source = /note="Description of Unknown: NRP-I4 sequence"
KYNIANVFL

SEQ ID NO: 73 - protein, 9 aa, unidentified
  REGION 1..9: note = source = /note="Description of Unknown: NRP-V7 sequence"
KYNKANVFL

SEQ ID NO: 74 - protein, 9 aa, unidentified
  REGION 1..9: note = source = /note="Description of Unknown: YAI/Db sequence"
FQDENYLYL

SEQ ID NO: 75 - protein, 9 aa, unidentified
  REGION 1..9: note = source = /note="Description of Unknown: INS B15-23 sequence"
LYLVCGERG

SEQ ID NO: 76 - protein, 15 aa, unidentified
  REGION 1..15: note = source = /note="Description of Unknown: PPI76-90 (K88S) sequence"
SLQPLALEGSLQSRG

SEQ ID NO: 77 - protein, 13 aa, unidentified
  REGION 1..13: note = source = /note="Description of Unknown: IGRP13-25 sequence"
QHLQKDYRAYYTF

SEQ ID NO: 78 - protein, 13 aa, unidentified
  REGION 1..13: note = source = /note="Description of Unknown: GAD555-567 sequence"
NFFRMVISNPAAT

SEQ ID NO: 79 - protein, 13 aa, unidentified
  REGION 1..13: note = source = /note="Description of Unknown: GAD555-567(557I) sequence"
NFIRMVISNPAAT

SEQ ID NO: 80 - protein, 13 aa, unidentified
  REGION 1..13: note = source = /note="Description of Unknown: IGRP23-35 sequence"
YTFLNFMSNVGDP

SEQ ID NO: 81 - protein, 13 aa, unidentified
  REGION 1..13: note = source = /note="Description of Unknown: B24-C36 sequence"
FFYTPKTRREAED

SEQ ID NO: 82 - protein, 15 aa, unidentified
  REGION 1..15: note = source = /note="Description of Unknown: PPI76-90 sequence"
SLQPLALEGSLQKRG

SEQ ID NO: 83 - protein, 9 aa, unidentified
  REGION 1..9: note = source = /note="Description of Unknown: INS-I9 sequence"
LYLVCGERI

SEQ ID NO: 84 - protein, 9 aa, unidentified
  REGION 1..9: note = source = /note="Description of Unknown: TUM sequence"
KYQAVTTTL

SEQ ID NO: 85 - protein, 9 aa, unidentified
  REGION 1..9: note = source = /note="Description of Unknown: G6Pase sequence"
KYCLITIFL

SEQ ID NO: 86 - protein, 9 aa, unidentified
  REGION 1..9: note = source = /note="Description of Unknown: Pro-insulinL2-10 sequence"
ALWMRLLPL

SEQ ID NO: 87 - protein, 9 aa, unidentified
  REGION 1..9: note = source = /note="Description of Unknown: Pro-insulinL3-11 sequence"
LWMRLLPLL

SEQ ID NO: 88 - protein, 9 aa, unidentified
  REGION 1..9: note = source = /note="Description of Unknown: Pro-insulinL6-14 sequence"
RLLPLLALL

SEQ ID NO: 89 - protein, 10 aa, unidentified
  REGION 1..10: note = source = /note="Description of Unknown: Pro-insulinB5-14 sequence"
HLCGSHLVEA

SEQ ID NO: 90 - protein, 9 aa, unidentified
  REGION 1..9: note = source = /note="Description of Unknown: Pro-insulinB10-18 sequence"
HLVEALYLV

SEQ ID NO: 91 - protein, 9 aa, unidentified
  REGION 1..9: note = source = /note="Description of Unknown: Pro-insulinB14-22 sequence"
ALYLVCGER

SEQ ID NO: 92 - protein, 10 aa, unidentified
  REGION 1..10: note = source = /note="Description of Unknown: Pro-insulinB15-24 sequence"
LYLVCGERGF

SEQ ID NO: 93 - protein, 9 aa, unidentified
  REGION 1..9: note = source = /note="Description of Unknown: Pro-insulinB17-25 sequence"
LVCGERGFF

SEQ ID NO: 94 - protein, 10 aa, unidentified
  REGION 1..10: note = source = /note="Description of Unknown: Pro-insulinB18-27 sequence"
VCGERGFFYT

SEQ ID NO: 95 - protein, 8 aa, unidentified
  REGION 1..8: note = source = /note="Description of Unknown: Pro-insulinB20-27 sequence"
GERGFFYT

SEQ ID NO: 96 - protein, 9 aa, unidentified
  REGION 1..9: note = source = /note="Description of Unknown: Pro-insulinB21-29 sequence"
ERGFFYTPK

SEQ ID NO: 97 - protein, 9 aa, unidentified
  REGION 1..9: note = source = /note="Description of Unknown: Pro-insulinB25-C1 sequence"
FYTPKTRRE

SEQ ID NO: 98 - protein, 11 aa, unidentified
  REGION 1..11: note = source = /note="Description of Unknown: Pro-insulinB27-C5 sequence"
TPKTRREAEDL

SEQ ID NO: 99 - protein, 9 aa, unidentified
  REGION 1..9: note = source = /note="Description of Unknown: Pro-insulinC20-28 sequence"
SLQPLALEG

SEQ ID NO: 100 - protein, 9 aa, unidentified
  REGION 1..9: note = source = /note="Description of Unknown: Pro-insulinC25-33 sequence"
ALEGSLQKR

SEQ ID NO: 101 - protein, 10 aa, unidentified
  REGION 1..10: note = source = /note="Description of Unknown: Pro-insulinC29-A5 sequence"
SLQKRGIVEQ

SEQ ID NO: 102 - protein, 10 aa, unidentified
  REGION 1..10: note = source = /note="Description of Unknown: Pro-insulinA1-10 sequence"
GIVEQCCTSI

SEQ ID NO: 103 - protein, 9 aa, unidentified
  REGION 1..9: note = source = /note="Description of Unknown: Pro-insulinA2-10 sequence"
IVEQCCTSI

SEQ ID NO: 104 - protein, 9 aa, unidentified
  REGION 1..9: note = source = /note="Description of Unknown: Pro-insulinA12-20 sequence"
SLYQLENYC

SEQ ID NO: 105 - protein, 21 aa, unidentified
  REGION 1..21: note = source = /note="Description of Unknown: MOG35-55 sequence"
MEVGWYRSPFSRVVHLYRNGK

SEQ ID NO: 106 - protein, 20 aa, unidentified
  REGION 1..20: note = source = /note="Description of Unknown: MOG36-55 sequence"
EVGWYRSPFSRVVHLYRNGK

SEQ ID NO: 107 - protein, 9 aa, unidentified
  REGION 1..9: note = source = /note="Description of Unknown: MAG287-295 sequence"
SLLLELEEV

SEQ ID NO: 108 - protein, 9 aa, unidentified
  REGION 1..9: note = source = /note="Description of Unknown: MAG509-517 sequence"
LMWAKIGPV

SEQ ID NO: 109 - protein, 9 aa, unidentified
  REGION 1..9: note = source = /note="Description of Unknown: MAG556-564 sequence"
VLFSSDFRI

SEQ ID NO: 110 - protein, 9 aa, unidentified
  REGION 1..9: note = source = /note="Description of Unknown: MBP110-118 sequence"
SLSRFSWGA

SEQ ID NO: 111 - protein, 9 aa, unidentified
  REGION 1..9: note = source = /note="Description of Unknown: MOG114-122 sequence"
KVEDPFYWV

SEQ ID NO: 112 - protein, 10 aa, unidentified
  REGION 1..10: note = source = /note="Description of Unknown: MOG166-175 sequence"
RTFDPHFLRV

SEQ ID NO: 113 - protein, 9 aa, unidentified
  REGION 1..9: note = source = /note="Description of Unknown: MOG172-180 sequence"
FLRVPCWKI

SEQ ID NO: 114 - protein, 10 aa, unidentified
  REGION 1..10: note = source = /note="Description of Unknown: MOG179-188 sequence"
KITLFVIVPV

SEQ ID NO: 115 - protein, 9 aa, unidentified
  REGION 1..9: note = source = /note="Description of Unknown: MOG188-196 sequence"
VLGPLVALI

SEQ ID NO: 116 - protein, 9 aa, unidentified
  REGION 1..9: note = source = /note="Description of Unknown: MOG181-189 sequence"
TLFVIVPVL

SEQ ID NO: 117 - protein, 10 aa, unidentified
  REGION 1..10: note = source = /note="Description of Unknown: MOG205-214 sequence"
RLAGQFLEEL

SEQ ID NO: 118 - protein, 9 aa, unidentified
  REGION 1..9: note = source = /note="Description of Unknown: PLP80-88 sequence"
FLYGALLLA

SEQ ID NO: 119 - protein, 9 aa, unidentified
  REGION 1..9: note = source = /note="Description of Unknown: MAG287-295 sequence"
SLLLELEEV

SEQ ID NO: 120 - protein, 9 aa, unidentified
  REGION 1..9: note = source = /note="Description of Unknown: MAG509-517 sequence"
LMWAKIGPV

SEQ ID NO: 121 - protein, 9 aa, unidentified
  REGION 1..9: note = source = /note="Description of Unknown: MAG556-564 sequence"
VLFSSDFRI

SEQ ID NO: 122 - protein, 13 aa, unidentified
  REGION 1..13: note = source = /note="Description of Unknown: MOG97-109 sequence"
TCFFRDHSYQEEA

SEQ ID NO: 123 - protein, 13 aa, unidentified
  REGION 1..13: note = source = /note="Description of Unknown: MOG97-109(E107S) sequence"
TCFFRDHSYQEEA

SEQ ID NO: 124 - protein, 13 aa, unidentified
  REGION 1..13: note = source = /note="Description of Unknown: MOG97-109(E107S) sequence"
TCFFRDHSYQSEA

SEQ ID NO: 125 - protein, 13 aa, unidentified
  REGION 1..13: note = source = /note="Description of Unknown: MBP89-101 sequence"
VHFFKNIVTPRTP

SEQ ID NO: 126 - protein, 18 aa, unidentified
  REGION 1..18: note = source = /note="Description of Unknown: PLP175-192 sequence"
YIYFNTWTTCQSIAFPSK

SEQ ID NO: 127 - protein, 15 aa, unidentified
  REGION 1..15: note = source = /note="Description of Unknown: PLP94-108 sequence"
GAVRQIFGDYKTTIC

SEQ ID NO: 128 - protein, 13 aa, unidentified
  REGION 1..13: note = source = /note="Description of Unknown: MBP86-98 sequence"
PVVHFFKNIVTPR

SEQ ID NO: 129 - protein, 15 aa, unidentified
  REGION 1..15: note = source = /note="Description of Unknown: PLP54-68 sequence"
NYQDYEYLINVIHAF

SEQ ID NO: 130 - protein, 15 aa, unidentified
  REGION 1..15: note = source = /note="Description of Unknown: PLP249-263 sequence"
ATLVSLLTFMIAATY

SEQ ID NO: 131 - protein, 15 aa, unidentified
  REGION 1..15: note = source = /note="Description of Unknown: MOG156-170 sequence"
LVLLAVLPVLLLQIT

SEQ ID NO: 132 - protein, 15 aa, unidentified
  REGION 1..15: note = source = /note="Description of Unknown: MOG201-215 sequence"
FLRVPCWKITLFVIV

SEQ ID NO: 133 - protein, 15 aa, unidentified
  REGION 1..15: note = source = /note="Description of Unknown: MOG38-52 sequence"
RHPIRALVGDEVELP

SEQ ID NO: 134 - protein, 15 aa, unidentified
  REGION 1..15: note = source = /note="Description of Unknown: MOG203-217 sequence"
RVPCWKITLFVIVPV

SEQ ID NO: 135 - protein, 15 aa, unidentified
  REGION 1..15: note = source = /note="Description of Unknown: PLP250-264 sequence"
TLVSLLTFMIAATYN

SEQ ID NO: 136 - protein, 20 aa, unidentified
  REGION 1..20: note = source = /note="Description of Unknown: MPB13-32 sequence"
KYLATASTMDHARHGFLPRH

SEQ ID NO: 137 - protein, 17 aa, unidentified
  REGION 1..17: note = source = /note="Description of Unknown: MPB83-99 sequence"
ENPVVHFFKNIVTPRTP

SEQ ID NO: 138 - protein, 19 aa, unidentified
  REGION 1..19: note = source = /note="Description of Unknown: MPB111-129 sequence"
LSRFSWGAEGQRPGFGYGG

SEQ ID NO: 139 - protein, 12 aa, unidentified
  REGION 1..12: note = source = /note="Description of Unknown: aGlia57-68 sequence"
QLQPFPQPELPY

SEQ ID NO: 140 - protein, 11 aa, unidentified
  REGION 1..11: note = source = /note="Description of Unknown: aGlia62-72 sequence"
PQPELPYPQPE

SEQ ID NO: 141 - protein, 13 aa, unidentified
  REGION 1..13: note = source = /note="Description of Unknown: aGlia217-229 sequence"
SGEGSFQPSQQNP

SEQ ID NO: 142 - protein, 14 aa, unidentified
  REGION 1..14: note = source = /note="Description of Unknown: PDC-E2122-135 sequence"
GDLIAEVETDKATV

SEQ ID NO: 143 - protein, 14 aa, unidentified
  REGION 1..14: note = source = /note="Description of Unknown: PDC-E2249-262 sequence"
GDLLAEIETDKATI

SEQ ID NO: 144 - protein, 15 aa, unidentified
  REGION 1..15: note = source = /note="Description of Unknown: PDC-E2249-263 sequence"
GDLLAEIETDKATIG

SEQ ID NO: 145 - protein, 15 aa, unidentified
  REGION 1..15: note = source = /note="Description of Unknown: PDC-E2629-643 sequence"
AQWLAEFRKYLEKPI

SEQ ID NO: 146 - protein, 15 aa, unidentified
  REGION 1..15: note = source = /note="Description of Unknown: PDC-E272-86 sequence"
RLLLQLLGSPGRRYY

SEQ ID NO: 147 - protein, 15 aa, unidentified
  REGION 1..15: note = source = /note="Description of Unknown: PDC-E2353-367 sequence"
GRVFVSPLAKKLAVE

SEQ ID NO: 148 - protein, 15 aa, unidentified
  REGION 1..15: note = source = /note="Description of Unknown: PDC-E2422-436 sequence"
DIPISNIRRVIAQRL

SEQ ID NO: 149 - protein, 15 aa, unidentified
  REGION 1..15: note = source = /note="Description of Unknown: PDC-E2629-643 sequence"
AQWLAEFRKYLEKPI

SEQ ID NO: 150 - protein, 15 aa, unidentified
  REGION 1..15: note = source = /note="Description of Unknown: PDC-E280-94 sequence"
SPGRRYYSLPPHQKV

SEQ ID NO: 151 - protein, 15 aa, unidentified
  REGION 1..15: note = source = /note="Description of Unknown: PDC-E2353-367 sequence"
GRVFVSPLAKKLAVE

SEQ ID NO: 152 - protein, 15 aa, unidentified
  REGION 1..15: note = source = /note="Description of Unknown: PDC-E2535-549 sequence"
ETIANDVVSLATKAR

SEQ ID NO: 153 - protein, 14 aa, unidentified
  REGION 1..14: note = source = /note="Description of Unknown: DG1216-229 sequence"
GEIRTMNNFLDREI

SEQ ID NO: 154 - protein, 15 aa, unidentified
  REGION 1..15: note = source = /note="Description of Unknown: DG397-111 sequence"
FGIFVVDKNTGDINI

SEQ ID NO: 155 - protein, 15 aa, unidentified
  REGION 1..15: note = source = /note="Description of Unknown: DG3251-265 sequence"
CECNIKVKDVNDNFP

SEQ ID NO: 156 - protein, 15 aa, unidentified
  REGION 1..15: note = source = /note="Description of Unknown: DG3351-365 sequence"
NKAEFHQSVISRYRV

SEQ ID NO: 157 - protein, 15 aa, unidentified
  REGION 1..15: note = source = /note="Description of Unknown: DG3453-467 sequence"
DSTFIVNKTITAEVL

SEQ ID NO: 158 - protein, 15 aa, unidentified
  REGION 1..15: note = source = /note="Description of Unknown: DG3540-554 sequence"
SITTLNATSALLRAQ

SEQ ID NO: 159 - protein, 15 aa, unidentified
  REGION 1..15: note = source = /note="Description of Unknown: DG3280-294 sequence"
ILSSELLRFQVTDLD

SEQ ID NO: 160 - protein, 15 aa, unidentified
  REGION 1..15: note = source = /note="Description of Unknown: DG3326-340 sequence"
EGILKVVKALDYEQL

SEQ ID NO: 161 - protein, 15 aa, unidentified
  REGION 1..15: note = source = /note="Description of Unknown: DG3367-381 sequence"
STPVTIQVINVREGI

SEQ ID NO: 162 - protein, 15 aa, unidentified
  REGION 1..15: note = source = /note="Description of Unknown: DG313-27 sequence"
AIFVVVILVHGELRI

SEQ ID NO: 163 - protein, 15 aa, unidentified
  REGION 1..15: note = source = /note="Description of Unknown: DG3323-337 sequence"
RTNEGILKVVKALDY

SEQ ID NO: 164 - protein, 15 aa, unidentified
  REGION 1..15: note = source = /note="Description of Unknown: DG3438-452 sequence"
DSKTAEIKFVKNMNR

SEQ ID NO: 165 - protein, 15 aa, unidentified
  REGION 1..15: note = source = /note="Description of Unknown: DG148-62 sequence"
KREWIKFAAACREGE

SEQ ID NO: 166 - protein, 15 aa, unidentified
  REGION 1..15: note = source = /note="Description of Unknown: DG1206-222 sequence"
MFIINRNTGEIRTMN

SEQ ID NO: 167 - protein, 15 aa, unidentified
  REGION 1..15: note = source = /note="Description of Unknown: DG1363-377 sequence"
SQYKLKASAISVTVL

SEQ ID NO: 168 - protein, 15 aa, unidentified
  REGION 1..15: note = source = /note="Description of Unknown: DG13-17 sequence"
WSFFRVVAMLFIFLV

SEQ ID NO: 169 - protein, 15 aa, unidentified
  REGION 1..15: note = source = /note="Description of Unknown: DG1192-206 sequence"
SKIAFKIIRQEPSDS

SEQ ID NO: 170 - protein, 15 aa, unidentified
  REGION 1..15: note = source = /note="Description of Unknown: DG1326-340 sequence"
TNVGILKVVKPLDYE

SEQ ID NO: 171 - protein, 15 aa, unidentified
  REGION 1..15: note = source = /note="Description of Unknown: DG11-15 sequence"
MDWSFFRVVAMLFIF

SEQ ID NO: 172 - protein, 15 aa, unidentified
  REGION 1..15: note = source = /note="Description of Unknown: DG135-49 sequence"
KNGTIKWHSIRRQKR

SEQ ID NO: 173 - protein, 15 aa, unidentified
  REGION 1..15: note = source = /note="Description of Unknown: DG1325-339 sequence"
RTNVGILKVVKPLDY

SEQ ID NO: 174 - protein, 15 aa, unidentified
  REGION 1..15: note = source = /note="Description of Unknown: AQP4129-143 sequence"
GAGILYLVTPPSVVG

SEQ ID NO: 175 - protein, 15 aa, unidentified
  REGION 1..15: note = source = /note="Description of Unknown: AQP4284-298 sequence"
RSQVETDDLILKPGV

SEQ ID NO: 176 - protein, 14 aa, unidentified
  REGION 1..14: note = source = /note="Description of Unknown: AQP463-76 sequence"
EKPLPVDMVLISLC

SEQ ID NO: 177 - protein, 15 aa, unidentified
  REGION 1..15: note = source = /note="Description of Unknown: AQP4129-143 sequence"
GAGILYLVTPPSVVG

SEQ ID NO: 178 - protein, 15 aa, unidentified
  REGION 1..15: note = source = /note="Description of Unknown: AQP439-53 sequence"
TAEFLAMLIFVLLSL

SEQ ID NO: 179 - protein, 15 aa, unidentified
  REGION 1..15: note = source = /note="Description of Unknown: DERP-116-30 sequence"
LRQMRTVTPIRMQGG

SEQ ID NO: 180 - protein, 15 aa, unidentified
  REGION 1..15: note = source = /note="Description of Unknown: DERP-1171-185 sequence"
AVNIVGYSNAQGVDY

SEQ ID NO: 181 - protein, 15 aa, unidentified
  REGION 1..15: note = source = /note="Description of Unknown: DERP-1110-124 sequence"
RFGISNYCQIYPPNV

SEQ ID NO: 182 - protein, 15 aa, unidentified
  REGION 1..15: note = source = /note="Description of Unknown: DERP-226-40 sequence"
PCIIHRGKPFQLEAV

SEQ ID NO: 183 - protein, 15 aa, unidentified
  REGION 1..15: note = source = /note="Description of Unknown: DERP-2107-121 sequence"
TVKVMGDDGVLACAI

SEQ ID NO: 184 - protein, 15 aa, Bacteroides sp.
EAINQGYMHADAYPF

SEQ ID NO: 185 - protein, 15 aa, Bacteroides sp.
KDLTYTFLRDFEQYL

SEQ ID NO: 186 - protein, 15 aa, Bacteroides sp.
RQLRTLVNEAINQGY

SEQ ID NO: 187 - protein, 15 aa, Bacteroides sp.
MDKIRYRLVYNRQNT

SEQ ID NO: 188 - protein, 15 aa, Bacteroides sp.
EAINQGYMHADAYPF

SEQ ID NO: 189 - protein, 15 aa, Bacteroides sp.
LNQRKIYLKTNVYLK

SEQ ID NO: 190 - protein, 15 aa, Bacteroides sp.
EYILYLQGIELGYWK

SEQ ID NO: 191 - protein, 15 aa, Bacteroides sp.
TCATLLIHQGVAITT

SEQ ID NO: 192 - protein, 15 aa, Bacteroides sp.
AKHMRQLRTLVNEAI

SEQ ID NO: 193 - protein, 15 aa, Bacteroides sp.
IRYRLVYNRQNTLNR

SEQ ID NO: 194 - protein, 15 aa, Bacteroides sp.
ENFIRINGKRWLYFK

SEQ ID NO: 195 - protein, 15 aa, unidentified
  REGION 1..15: note = source = /note="Description of Unknown: Fla-2/Fla-X366-380 sequence"
TGAAATYAIDSIADA

SEQ ID NO: 196 - protein, 15 aa, unidentified
  REGION 1..15: note = source = /note="Description of Unknown: Fla-2/Fla-X164-178 sequence"
NATFSMDQLKFGDTI

SEQ ID NO: 197 - protein, 15 aa, unidentified
  REGION 1..15: note = source = /note="Description of Unknown: Fla-2/Fla-X261-275 sequence"
DRTVVSSIGAYKLIQ

SEQ ID NO: 198 - protein, 15 aa, unidentified
  REGION 1..15: note = source = /note="Description of Unknown: Fla-2/Fla-X1-15 sequence"
MVVQHNLRAMNSNRM

SEQ ID NO: 199 - protein, 15 aa, unidentified
  REGION 1..15: note = source = /note="Description of Unknown: Fla-2/Fla-X51-65 sequence"
KMRKQIRGLSQASLN

SEQ ID NO: 200 - protein, 15 aa, unidentified
  REGION 1..15: note = source = /note="Description of Unknown: Fla-2/Fla-X269-283 sequence"
GAYKLIQKELGLASS

SEQ ID NO: 201 - protein, 15 aa, unidentified
  REGION 1..15: note = source = /note="Description of Unknown: Fla-2/Fla-X4-18 sequence"
QHNLRAMNSNRMLGI

SEQ ID NO: 202 - protein, 15 aa, unidentified
  REGION 1..15: note = source = /note="Description of Unknown: Fla-2/Fla-X271-285 sequence"
YKLIQKELGLASSIG

SEQ ID NO: 203 - protein, 15 aa, Escherichia coli
ADDIVKMLNDPALNR

SEQ ID NO: 204 - protein, 15 aa, Escherichia coli
HNIQVADDARFVLNA

SEQ ID NO: 205 - protein, 15 aa, Escherichia coli
ADDARFVLNAGKKKF

SEQ ID NO: 206 - protein, 15 aa, Escherichia coli
GCISYALVSHTAKGS

SEQ ID NO: 207 - protein, 15 aa, Escherichia coli
ADDIVKMLNDPALNR

SEQ ID NO: 208 - protein, 15 aa, Escherichia coli
LPVTVTLDIITAPLQ

SEQ ID NO: 209 - protein, 15 aa, Escherichia coli
SGCISYALVSHTAKG

SEQ ID NO: 210 - protein, 15 aa, Escherichia coli
DIVKMLNDPALNRHN

SEQ ID NO: 211 - protein, 15 aa, Escherichia coli
ARFVLNAGKKKFTGT

SEQ ID NO: 212 - protein, 24 aa, unidentified
  REGION 1..24: note = source = /note="Description of Unknown: H471-94 sequence"
TYTEHAKRKTVTAMDVVYALKRQG

SEQ ID NO: 213 - protein, 15 aa, unidentified
  REGION 1..15: note = source = /note="Description of Unknown: H474-88 sequence"
EHAKRKTVTAMDVVY

SEQ ID NO: 214 - protein, 15 aa, unidentified
  REGION 1..15: note = source = /note="Description of Unknown: H476-90 sequence"
AKRKTVTAMDVVYAL

SEQ ID NO: 215 - protein, 15 aa, unidentified
  REGION 1..15: note = source = /note="Description of Unknown: H475-89 sequence"
HAKRKTVTAMDVVYA

SEQ ID NO: 216 - protein, 15 aa, unidentified
  REGION 1..15: note = source = /note="Description of Unknown: H478-92 sequence"
RKTVTAMDVVYALKR

SEQ ID NO: 217 - protein, 14 aa, unidentified
  REGION 1..14: note = source = /note="Description of Unknown: H480-94 sequence"
TVTAMDVVYALKRQ

SEQ ID NO: 218 - protein, 15 aa, unidentified
  REGION 1..15: note = source = /note="Description of Unknown: H2B10-24 sequence"
PKKGSKKAVTKAQKK

SEQ ID NO: 219 - protein, 15 aa, unidentified
  REGION 1..15: note = source = /note="Description of Unknown: H2B16-30 sequence"
KAVTKAQKKDGKKRK

SEQ ID NO: 220 - protein, 21 aa, unidentified
  REGION 1..21: note = source = /note="Description of Unknown: H1'22-42 sequence"
STDHPKYSDMIVAAIQAEKNR

SEQ ID NO: 221 - protein, 15 aa, unidentified
  REGION 1..15: note = source = /note="Description of Unknown: H1'27-41 sequence"
KYSDMIVAAIQAEKN

SEQ ID NO: 222 - protein, 15 aa, unidentified
  REGION 1..15: note = source = /note="Description of Unknown: ApoB3501-3516 sequence"
SQEYSGSVANEANVY

SEQ ID NO: 223 - protein, 15 aa, unidentified
  REGION 1..15: note = source = /note="Description of Unknown: ApoB1952-1966 sequence"
SHSLPYESSISTALE

SEQ ID NO: 224 - protein, 15 aa, unidentified
  REGION 1..15: note = source = /note="Description of Unknown: ApoB978-993 sequence"
TGAYSNASSTESASY

SEQ ID NO: 225 - protein, 15 aa, unidentified
  REGION 1..15: note = source = /note="Description of Unknown: ApoB3498-3513 sequence"
SFLSQEYSGSVANEA

SEQ ID NO: 226 - protein, 20 aa, unidentified
  REGION 1..20: note = source = /note="Description of Unknown: ApoB210A sequence"
KTTKQSFDLSVKAQYKKNKH

SEQ ID NO: 227 - protein, 15 aa, unidentified
  REGION 1..15: note = source = /note="Description of Unknown: ApoB210B sequence"
KTTKQSFDLSVKAQY

SEQ ID NO: 228 - protein, 15 aa, unidentified
  REGION 1..15: note = source = /note="Description of Unknown: ApoB210C sequence"
TTKQSFDLSVKAQYK

SEQ ID NO: 229 - protein, 15 aa, unidentified
  REGION 1..15: note = source = /note="Description of Unknown: elastin89-103 sequence"
GALVPGGVADAAAAY

SEQ ID NO: 230 - protein, 15 aa, unidentified
  REGION 1..15: note = source = /note="Description of Unknown: elastin698-712 sequence"
AAQFGLVGAAGLGGL

SEQ ID NO: 231 - protein, 15 aa, unidentified
  REGION 1..15: note = source = /note="Description of Unknown: elastin8-22 sequence"
APRPGVLLLLLSILH

SEQ ID NO: 232 - protein, 15 aa, unidentified
  REGION 1..15: note = source = /note="Description of Unknown: elastin94-108 sequence"
GGVADAAAAYKAAKA

SEQ ID NO: 233 - protein, 15 aa, unidentified
  REGION 1..15: note = source = /note="Description of Unknown: elastin13-27 sequence"
VLLLLLSILHPSRPG

SEQ ID NO: 234 - protein, 15 aa, unidentified
  REGION 1..15: note = source = /note="Description of Unknown: elastin695-709 sequence"
AAKAAQFGLVGAAGL

SEQ ID NO: 235 - protein, 15 aa, unidentified
  REGION 1..15: note = source = /note="Description of Unknown: elastin563-577 sequence"
VAAKAQLRAAAGLGA

SEQ ID NO: 236 - protein, 15 aa, unidentified
  REGION 1..15: note = source = /note="Description of Unknown: elastin558-572 sequence"
KSAAKVAAKAQLRAA

SEQ ID NO: 237 - protein, 15 aa, unidentified
  REGION 1..15: note = source = /note="Description of Unknown: elastin698-712 sequence"
AAQFGLVGAAGLGGL

SEQ ID NO: 238 - protein, 15 aa, unidentified
  REGION 1..15: note = source = /note="Description of Unknown: elastin566-580 sequence"
KAQLRAAAGLGAGIP

SEQ ID NO: 239 - protein, 15 aa, unidentified
  REGION 1..15: note = source = /note="Description of Unknown: elastin645-659 sequence"
VPGALAAAKAAKYGA

SEQ ID NO: 240 - protein, 15 aa, unidentified
  REGION 1..15: note = source = /note="Description of Unknown: Cap1864-78 sequence"
RPTMDGDPDTPKPVS

SEQ ID NO: 241 - protein, 15 aa, unidentified
  REGION 1..15: note = source = /note="Description of Unknown: Cap1834-48 sequence"
SYKEAVLRAIDGINQ

SEQ ID NO: 242 - protein, 15 aa, unidentified
  REGION 1..15: note = source = /note="Description of Unknown: Cap1847-61 sequence"
NQRSSDANLYRLLDL

SEQ ID NO: 243 - protein, 15 aa, unidentified
  REGION 1..15: note = source = /note="Description of Unknown: Cap18151-165 sequence"
KRIVQRIKDFLRNLV

SEQ ID NO: 244 - protein, 15 aa, unidentified
  REGION 1..15: note = source = /note="Description of Unknown: Cap18149-163 sequence"
EFKRIVQRIKDFLRN

SEQ ID NO: 245 - protein, 15 aa, unidentified
  REGION 1..15: note = source = /note="Description of Unknown: Cap18152-166 sequence"
RIVQRIKDFLRNLVP

SEQ ID NO: 246 - protein, 15 aa, unidentified
  REGION 1..15: note = source = /note="Description of Unknown: Cap18131-145 sequence"
RFALLGDFFRKSKEK

SEQ ID NO: 247 - protein, 15 aa, unidentified
  REGION 1..15: note = source = /note="Description of Unknown: Cap1824-38 sequence"
QRIKDFLRNLVPRTE

SEQ ID NO: 248 - protein, 15 aa, unidentified
  REGION 1..15: note = source = /note="Description of Unknown: ADMTSL5245-259 sequence"
DGRYVLNGHWVVSPP

SEQ ID NO: 249 - protein, 15 aa, unidentified
  REGION 1..15: note = source = /note="Description of Unknown: ADMTSL5267-281 sequence"
THVVYTRDTGPQETL

SEQ ID NO: 250 - protein, 15 aa, unidentified
  REGION 1..15: note = source = /note="Description of Unknown: ADMTSL5372-386 sequence"
RLLHYCGSDFVFQAR

SEQ ID NO: 251 - protein, 15 aa, unidentified
  REGION 1..15: note = source = /note="Description of Unknown: ADMTSL5289-303 sequence"
HDLLLQVLLQEPNPG

SEQ ID NO: 252 - protein, 15 aa, unidentified
  REGION 1..15: note = source = /note="Description of Unknown: ADMTSL5396-410 sequence"
ETRYEVRIQLVYKNR

SEQ ID NO: 253 - protein, 15 aa, unidentified
  REGION 1..15: note = source = /note="Description of Unknown: ADMTSL5433-447 sequence"
HRDYLMAVQRLVSPD

SEQ ID NO: 254 - protein, 15 aa, unidentified
  REGION 1..15: note = source = /note="Description of Unknown: ADMTSL5142-156 sequence"
EGHAFYHSFGRVLDG

SEQ ID NO: 255 - protein, 15 aa, unidentified
  REGION 1..15: note = source = /note="Description of Unknown: ADMTSL5236-250 sequence"
RNHLALMGGDGRYVL

SEQ ID NO: 256 - protein, 15 aa, unidentified
  REGION 1..15: note = source = /note="Description of Unknown: ADMTSL5301-315 sequence"
NPGIEFEFWLPRERY

SEQ ID NO: 257 - protein, 15 aa, unidentified
  REGION 1..15: note = source = /note="Description of Unknown: ADMTSL5203-217 sequence"
VQRVFRDAGAFAGYW

SEQ ID NO: 258 - protein, 15 aa, unidentified
  REGION 1..15: note = source = /note="Description of Unknown: ADMTSL5404-418 sequence"
QLVYKNRSPLRAREY

SEQ ID NO: 259 - protein, 15 aa, unidentified
  REGION 1..15: note = source = /note="Description of Unknown: CYP2D6193-207 sequence"
RRFEYDDPRFLRLLD

SEQ ID NO: 260 - protein, 15 aa, unidentified
  REGION 1..15: note = source = /note="Description of Unknown: CYP2D676-90 sequence"
TPVVVLNGLAAVREA

SEQ ID NO: 261 - protein, 15 aa, unidentified
  REGION 1..15: note = source = /note="Description of Unknown: CYP2D6293-307 sequence"
ENLRIVVADLFSAGM

SEQ ID NO: 262 - protein, 20 aa, unidentified
  REGION 1..20: note = source = /note="Description of Unknown: CYP2D6313-332 sequence"
TLAWGLLLMILHPDVQRRVQ

SEQ ID NO: 263 - protein, 20 aa, unidentified
  REGION 1..20: note = source = /note="Description of Unknown: CYP2D6393-412 sequence"
TTLITNLSSVLKDEAVWEKP

SEQ ID NO: 264 - protein, 15 aa, unidentified
  REGION 1..15: note = source = /note="Description of Unknown: CYP2D6199-213 sequence"
DPRFLRLLDLAQEGL

SEQ ID NO: 265 - protein, 15 aa, unidentified
  REGION 1..15: note = source = /note="Description of Unknown: CYP2D6450-464 sequence"
RMELFLFFTSLLQHF

SEQ ID NO: 266 - protein, 15 aa, unidentified
  REGION 1..15: note = source = /note="Description of Unknown: CYP2D6301-315 sequence"
DLFSAGMVTTSTTLA

SEQ ID NO: 267 - protein, 15 aa, unidentified
  REGION 1..15: note = source = /note="Description of Unknown: CYP2D6452-466 sequence"
ELFLFFTSLLQHFSF

SEQ ID NO: 268 - protein, 15 aa, unidentified
  REGION 1..15: note = source = /note="Description of Unknown: CYP2D659-73 sequence"
DQLRRRFGDVFSLQL

SEQ ID NO: 269 - protein, 15 aa, unidentified
  REGION 1..15: note = source = /note="Description of Unknown: CYP2D6130-144 sequence"
EQRRFSVSTLRNLGL

SEQ ID NO: 270 - protein, 20 aa, unidentified
  REGION 1..20: note = source = /note="Description of Unknown: CYP2D6193-212 sequence"
RRFEYDDPRFLRLLDLAQEG

SEQ ID NO: 271 - protein, 20 aa, unidentified
  REGION 1..20: note = source = /note="Description of Unknown: CYP2D6305-324 sequence"
AGMVTTSTTLAWGLLLMILH

SEQ ID NO: 272 - protein, 15 aa, unidentified
  REGION 1..15: note = source = /note="Description of Unknown: CYP2D6131-145 sequence"
QRRFSVSTLRNLGLG

SEQ ID NO: 273 - protein, 15 aa, unidentified
  REGION 1..15: note = source = /note="Description of Unknown: CYP2D6216-230 sequence"
ESGFLREVLNAVPVL

SEQ ID NO: 274 - protein, 15 aa, unidentified
  REGION 1..15: note = source = /note="Description of Unknown: CYP2D6238-252 sequence"
GKVLRFQKAFLTQLD

SEQ ID NO: 275 - protein, 15 aa, unidentified
  REGION 1..15: note = source = /note="Description of Unknown: CYP2D6199-213 sequence"
DPRFLRLLDLAQEGL

SEQ ID NO: 276 - protein, 15 aa, unidentified
  REGION 1..15: note = source = /note="Description of Unknown: CYP2D6235-252 sequence"
GKVLRFQKAFLTQLD

SEQ ID NO: 277 - protein, 15 aa, unidentified
  REGION 1..15: note = source = /note="Description of Unknown: CYP2D6293-307 sequence"
ENLRIVVADLFSAGM

SEQ ID NO: 278 - protein, 15 aa, unidentified
  REGION 1..15: note = source = /note="Description of Unknown: CYP2D6381-395 sequence"
DIEVQGFRIPKGTTL

SEQ ID NO: 279 - protein, 15 aa, unidentified
  REGION 1..15: note = source = /note="Description of Unknown: CYP2D6429-443 sequence"
KPEAFLPFSAGRRAC

SEQ ID NO: 280 - protein, 15 aa, unidentified
  REGION 1..15: note = source = /note="Description of Unknown: SLA334-348 sequence"
YKKLLKERKEMFSYL

SEQ ID NO: 281 - protein, 15 aa, unidentified
  REGION 1..15: note = source = /note="Description of Unknown: SLA 196-210 sequence"
DELRTDLKAVEAKVQ

SEQ ID NO: 282 - protein, 15 aa, unidentified
  REGION 1..15: note = source = /note="Description of Unknown: SLA115-129 sequence"
NKITNSLVLDIIKLA

SEQ ID NO: 283 - protein, 14 aa, unidentified
  REGION 1..14: note = source = /note="Description of Unknown: SLA 373-386 sequence"
NRLDRCLKAVRKER

SEQ ID NO: 284 - protein, 12 aa, unidentified
  REGION 1..12: note = source = /note="Description of Unknown: SLA 186-197 sequence"
LIQQGARVGRID

SEQ ID NO: 285 - protein, 15 aa, unidentified
  REGION 1..15: note = source = /note="Description of Unknown: SLA 317-331 sequence"
SPSLDVLITLLSLGS

SEQ ID NO: 286 - protein, 15 aa, unidentified
  REGION 1..15: note = source = /note="Description of Unknown: SLA 171-185 sequence"
DQKSCFKSMITAGFE

SEQ ID NO: 287 - protein, 15 aa, unidentified
  REGION 1..15: note = source = /note="Description of Unknown: SLA 417-431 sequence"
YTFRGFMSHTNNYPC

SEQ ID NO: 288 - protein, 15 aa, unidentified
  REGION 1..15: note = source = /note="Description of Unknown: SLA 359-373 sequence"
YNERLLHTPHNPISL

SEQ ID NO: 289 - protein, 15 aa, unidentified
  REGION 1..15: note = source = /note="Description of Unknown: SLA 215-229 sequence"
DCILCIHSTTSCFAP

SEQ ID NO: 290 - protein, 15 aa, unidentified
  REGION 1..15: note = source = /note="Description of Unknown: SLA111-125 sequence"
SSLLNKITNSLVLDI

SEQ ID NO: 291 - protein, 15 aa, unidentified
  REGION 1..15: note = source = /note="Description of Unknown: SLA110-124 sequence"
GSSLLNKITNSLVLD

SEQ ID NO: 292 - protein, 15 aa, unidentified
  REGION 1..15: note = source = /note="Description of Unknown: SLA299-313 sequence"
NDSFIQEISKMYPGR

SEQ ID NO: 293 - protein, 15 aa, unidentified
  REGION 1..15: note = source = /note="Description of Unknown: SLA342-356 sequence"
KEMFSYLSNQIKKLS

SEQ ID NO: 294 - protein, 15 aa, unidentified
  REGION 1..15: note = source = /note="Description of Unknown: SLA49-63 sequence"
STLELFLHELAIMDS

SEQ ID NO: 295 - protein, 15 aa, unidentified
  REGION 1..15: note = source = /note="Description of Unknown: SLA119-133 sequence"
NSLVLDIIKLAGVHT

SEQ ID NO: 296 - protein, 15 aa, unidentified
  REGION 1..15: note = source = /note="Description of Unknown: SLA260-274 sequence"
SKCMHLIQQGARVGR

SEQ ID NO: 297 - protein, 15 aa, unidentified
  REGION 1..15: note = source = /note="Description of Unknown: SLA26-40 sequence"
RSHEHLIRLLLEKGK

SEQ ID NO: 298 - protein, 15 aa, unidentified
  REGION 1..15: note = source = /note="Description of Unknown: SLA86-100 sequence"
RRHYRFIHGIGRSGD

SEQ ID NO: 299 - protein, 15 aa, unidentified
  REGION 1..15: note = source = /note="Description of Unknown: SLA331-345 sequence"
SNGYKKLLKERKEMF

SEQ ID NO: 300 - protein, 16 aa, unidentified
  REGION 1..16: note = source = /note="Description of Unknown: arrestin199-213 sequence"
QFFMSDKPLHLAVSLN

SEQ ID NO: 301 - protein, 15 aa, unidentified
  REGION 1..15: note = source = /note="Description of Unknown: arrestin77-91 sequence"
DVIGLTFRRDLYFSR

SEQ ID NO: 302 - protein, 15 aa, unidentified
  REGION 1..15: note = source = /note="Description of Unknown: arrestin250-264 sequence"
NVVLYSSDYYVKPVA

SEQ ID NO: 303 - protein, 15 aa, unidentified
  REGION 1..15: note = source = /note="Description of Unknown: arrestin172-186 sequence"
SSVRLLIRKVQHAPL

SEQ ID NO: 304 - protein, 15 aa, unidentified
  REGION 1..15: note = source = /note="Description of Unknown: arrestin354-368 sequence"
EVPFRLMHPQPEDPA

SEQ ID NO: 305 - protein, 15 aa, unidentified
  REGION 1..15: note = source = /note="Description of Unknown: arrestin239-253 sequence"
KKIKAFVEQVANVVL

SEQ ID NO: 306 - protein, 15 aa, unidentified
  REGION 1..15: note = source = /note="Description of Unknown: arrestin102-116 sequence"
STPTKLQESLLKKLG

SEQ ID NO: 307 - protein, 15 aa, unidentified
  REGION 1..15: note = source = /note="Description of Unknown: arrestin59-73 sequence"
KKVYVTLTCAFRYGQ

SEQ ID NO: 308 - protein, 15 aa, unidentified
  REGION 1..15: note = source = /note="Description of Unknown: arrestin280-294 sequence"
KTLTLLPLLANNRER

SEQ ID NO: 309 - protein, 16 aa, unidentified
  REGION 1..16: note = source = /note="Description of Unknown: arrestin291-306 sequence"
NRERRGIALDGKIKHE

SEQ ID NO: 310 - protein, 15 aa, unidentified
  REGION 1..15: note = source = /note="Description of Unknown: arrestin195-209 sequence"
EAAWQFFMSDKPLHL

SEQ ID NO: 311 - protein, 15 aa, unidentified
  REGION 1..15: note = source = /note="Description of Unknown: arrestin200-214 sequence"
QFFMSDKPLHLAVSL

SEQ ID NO: 312 - protein, 15 aa, unidentified
  REGION 1..15: note = source = /note="Description of Unknown: RO60127-141 sequence"
TFIQFKKDLKESMKC

SEQ ID NO: 313 - protein, 15 aa, unidentified
  REGION 1..15: note = source = /note="Description of Unknown: RO60523-537 sequence"
DTGALDVIRNFTLDM

SEQ ID NO: 314 - protein, 15 aa, unidentified
  REGION 1..15: note = source = /note="Description of Unknown: RO60243-257 sequence"
EVIHLIEEHRLVREH

SEQ ID NO: 315 - protein, 15 aa, unidentified
  REGION 1..15: note = source = /note="Description of Unknown: RO60484-498 sequence"
REYRKKMDIPAKLIV

SEQ ID NO: 316 - protein, 15 aa, unidentified
  REGION 1..15: note = source = /note="Description of Unknown: RO60347-361 sequence"
EEILKALDAAFYKTF

SEQ ID NO: 317 - protein, 15 aa, unidentified
  REGION 1..15: note = source = /note="Description of Unknown: RO60369-383 sequence"
KRFLLAVDVSASMNQ

SEQ ID NO: 318 - protein, 15 aa, unidentified
  REGION 1..15: note = source = /note="Description of Unknown: RO60426-440 sequence"
TDMTLQQVLMAMSQI

SEQ ID NO: 319 - protein, 15 aa, unidentified
  REGION 1..15: note = source = /note="Description of Unknown: RO60267-281 sequence"
EVWKALLQEMPLTAL

SEQ ID NO: 320 - protein, 15 aa, unidentified
  REGION 1..15: note = source = /note="Description of Unknown: RO60178-192 sequence"
SHKDLLRLSHLKPSS

SEQ ID NO: 321 - protein, 15 aa, unidentified
  REGION 1..15: note = source = /note="Description of Unknown: RO60358-372 sequence"
YKTFKTVEPTGKRFL

SEQ ID NO: 322 - protein, 15 aa, unidentified
  REGION 1..15: note = source = /note="Description of Unknown: RO60221-235 sequence"
ETEKLLKYLEAVEKV

SEQ ID NO: 323 - protein, 15 aa, unidentified
  REGION 1..15: note = source = /note="Description of Unknown: RO60318-332 sequence"
RIHPFHILIALETYK

SEQ ID NO: 324 - protein, 15 aa, unidentified
  REGION 1..15: note = source = /note="Description of Unknown: RO60407-421 sequence"
EKDSYVVAFSDEMVP

SEQ ID NO: 325 - protein, 15 aa, unidentified
  REGION 1..15: note = source = /note="Description of Unknown: RO60459-473 sequence"
TPADVFIVFTDNETF

SEQ ID NO: 326 - protein, 15 aa, unidentified
  REGION 1..15: note = source = /note="Description of Unknown: RO6051-65 sequence"
QKLGLENAEALIRLI

SEQ ID NO: 327 - protein, 15 aa, unidentified
  REGION 1..15: note = source = /note="Description of Unknown: RO60312-326 sequence"
KLLKKARIHPFHILI

SEQ ID NO: 328 - protein, 15 aa, unidentified
  REGION 1..15: note = source = /note="Description of Unknown: LA241-255 sequence"
DDQTCREDLHILFSN

SEQ ID NO: 329 - protein, 15 aa, unidentified
  REGION 1..15: note = source = /note="Description of Unknown: LA101-115 sequence"
TDEYKNDVKNRSVYI

SEQ ID NO: 330 - protein, 15 aa, unidentified
  REGION 1..15: note = source = /note="Description of Unknown: LA153-167 sequence"
SIFVVFDSIESAKKF

SEQ ID NO: 331 - protein, 15 aa, unidentified
  REGION 1..15: note = source = /note="Description of Unknown: LA178-192 sequence"
TDLLILFKDDYFAKK

SEQ ID NO: 332 - protein, 15 aa, unidentified
  REGION 1..15: note = source = /note="Description of Unknown: LA19-33 sequence"
HQIEYYFGDFNLPRD

SEQ ID NO: 333 - protein, 15 aa, unidentified
  REGION 1..15: note = source = /note="Description of Unknown: LA37-51 sequence"
KEQIKLDEGWVPLEI

SEQ ID NO: 334 - protein, 15 aa, unidentified
  REGION 1..15: note = source = /note="Description of Unknown: LA133-147 sequence"
DKGQVLNIQMRRTLH

SEQ ID NO: 335 - protein, 15 aa, unidentified
  REGION 1..15: note = source = /note="Description of Unknown: LA50-64 sequence"
EIMIKFNRLNRLTTD

SEQ ID NO: 336 - protein, 15 aa, unidentified
  REGION 1..15: note = source = /note="Description of Unknown: LA32-46 sequence"
RDKFLKEQIKLDEGW

SEQ ID NO: 337 - protein, 15 aa, unidentified
  REGION 1..15: note = source = /note="Description of Unknown: LA153-167 sequence"
SIFVVFDSIESAKKF

SEQ ID NO: 338 - protein, 15 aa, unidentified
  REGION 1..15: note = source = /note="Description of Unknown: LA83-97 sequence"
SEDKTKIRRSPSKPL

SEQ ID NO: 339 - protein, 15 aa, unidentified
  REGION 1..15: note = source = /note="Description of Unknown: LA136-150 sequence"
QVLNIQMRRTLHKAF

SEQ ID NO: 340 - protein, 15 aa, unidentified
  REGION 1..15: note = source = /note="Description of Unknown: LA297-311 sequence"
RNKEVTWEVLEGEVE

SEQ ID NO: 341 - protein, 15 aa, unidentified
  REGION 1..15: note = source = /note="Description of Unknown: LA59-73 sequence"
NRLTTDFNVIVEALS

SEQ ID NO: 342 - protein, 15 aa, unidentified
  REGION 1..15: note = source = /note="Description of Unknown: LA151-165 sequence"
KGSIFVVFDSIESAK

SEQ ID NO: 343 - protein, 15 aa, unidentified
  REGION 1..15: note = source = /note="Description of Unknown: LA86-100 sequence"
KTKIRRSPSKPLPEV

SEQ ID NO: 344 - protein, 15 aa, unidentified
  REGION 1..15: note = source = /note="Description of Unknown: LA154-168 sequence"
IFVVFDSIESAKKFV

SEQ ID NO: 345 - protein, 15 aa, unidentified
  REGION 1..15: note = source = /note="Description of Unknown: TOP1346-360 sequence"
KERIANFKIEPPGLF

SEQ ID NO: 346 - protein, 15 aa, unidentified
  REGION 1..15: note = source = /note="Description of Unknown: TOP1420-434 sequence"
QGSIKYIMLNPSSRI

SEQ ID NO: 347 - protein, 15 aa, unidentified
  REGION 1..15: note = source = /note="Description of Unknown: TOP1750-764 sequence"
QREKFAWAIDMADED

SEQ ID NO: 348 - protein, 15 aa, unidentified
  REGION 1..15: note = source = /note="Description of Unknown: TOP1419-433 sequence"
IQGSIKYIMLNPSSR

SEQ ID NO: 349 - protein, 15 aa, unidentified
  REGION 1..15: note = source = /note="Description of Unknown: TOP1591-605 sequence"
YNASITLQQQLKELT

SEQ ID NO: 350 - protein, 15 aa, unidentified
  REGION 1..15: note = source = /note="Description of Unknown: TOP1695-709 sequence"
EQLMKLEVQATDREE

SEQ ID NO: 351 - protein, 15 aa, unidentified
  REGION 1..15: note = source = /note="Description of Unknown: TOP1305-319 sequence"
SQYFKAQTEARKQMS

SEQ ID NO: 352 - protein, 15 aa, unidentified
  REGION 1..15: note = source = /note="Description of Unknown: TOP1346-360 sequence"
KERIANFKIEPPGLF

SEQ ID NO: 353 - protein, 15 aa, unidentified
  REGION 1..15: note = source = /note="Description of Unknown: TOP1419-433 sequence"
IQGSIKYIMLNPSSR

SEQ ID NO: 354 - protein, 15 aa, unidentified
  REGION 1..15: note = source = /note="Description of Unknown: TOP1425-439 sequence"
YIMLNPSSRIKGEKD

SEQ ID NO: 355 - protein, 15 aa, unidentified
  REGION 1..15: note = source = /note="Description of Unknown: TOP1614-628 sequence"
KILSYNRANRAVAIL

SEQ ID NO: 356 - protein, 15 aa, unidentified
  REGION 1..15: note = source = /note="Description of Unknown: CENP-C297-311 sequence"
KLIEDEFIIDESDQS

SEQ ID NO: 357 - protein, 15 aa, unidentified
  REGION 1..15: note = source = /note="Description of Unknown: CENP-C857-871 sequence"
KVYKTLDTPFFSTGK

SEQ ID NO: 358 - protein, 15 aa, unidentified
  REGION 1..15: note = source = /note="Description of Unknown: CENP-C887-901 sequence"
QDILVFYVNFGDLLC

SEQ ID NO: 359 - protein, 15 aa, unidentified
  REGION 1..15: note = source = /note="Description of Unknown: CENP-C212-226 sequence"
KVMLKKIEIDNKVSD

SEQ ID NO: 360 - protein, 15 aa, unidentified
  REGION 1..15: note = source = /note="Description of Unknown: CENP-C643-657 sequence"
EDNIMTAQNVPLKPQ

SEQ ID NO: 361 - protein, 15 aa, unidentified
  REGION 1..15: note = source = /note="Description of Unknown: CENP-C832-846 sequence"
TREIILMDLVRPQDT

SEQ ID NO: 362 - protein, 15 aa, unidentified
  REGION 1..15: note = source = /note="Description of Unknown: CENP-C167-181 sequence"
TSVSQNVIPSSAQKR

SEQ ID NO: 363 - protein, 15 aa, unidentified
  REGION 1..15: note = source = /note="Description of Unknown: CENP-C246-260 sequence"
RIRDSEYEIQRQAKK

SEQ ID NO: 364 - protein, 15 aa, unidentified
  REGION 1..15: note = source = /note="Description of Unknown: CENP-C846-860 sequence"
TYQFFVKHGELKVYK

SEQ ID NO: 365 - protein, 15 aa, unidentified
  REGION 1..15: note = source = /note="Description of Unknown: CENP-C149-163 sequence"
DEEFYLSVGSPSVLL

SEQ ID NO: 366 - protein, 15 aa, unidentified
  REGION 1..15: note = source = /note="Description of Unknown: CENP-C833-847 sequence"
REIILMDLVRPQDTY

SEQ ID NO: 367 - protein, 15 aa, unidentified
  REGION 1..15: note = source = /note="Description of Unknown: CENP-C847-861 sequence"
YQFFVKHGELKVYKT

SEQ ID NO: 368 - protein, 15 aa, unidentified
  REGION 1..15: note = source = /note="Description of Unknown: APOH235-249 sequence"
HDGYSLDGPEEIECT

SEQ ID NO: 369 - protein, 15 aa, unidentified
  REGION 1..15: note = source = /note="Description of Unknown: APOH306-320 sequence"
KCSYTEDAQCIDGTI

SEQ ID NO: 370 - protein, 15 aa, unidentified
  REGION 1..15: note = source = /note="Description of Unknown: APOH237-251 sequence"
GYSLDGPEEIECTKL

SEQ ID NO: 371 - protein, 15 aa, unidentified
  REGION 1..15: note = source = /note="Description of Unknown: APOH295-309 sequence"
KVSFFCKNKEKKCSY

SEQ ID NO: 372 - protein, 15 aa, unidentified
  REGION 1..15: note = source = /note="Description of Unknown: APOH28-42 sequence"
DLPFSTVVPLKTFYE

SEQ ID NO: 373 - protein, 15 aa, unidentified
  REGION 1..15: note = source = /note="Description of Unknown: APOH173-187 sequence"
ECLPQHAMFGNDTIT

SEQ ID NO: 374 - protein, 15 aa, unidentified
  REGION 1..15: note = source = /note="Description of Unknown: APOH264-278 sequence"
CKVPVKKATVVYQGE

SEQ ID NO: 375 - protein, 15 aa, unidentified
  REGION 1..15: note = source = /note="Description of Unknown: APOH295-309 sequence"
KVSFFCKNKEKKCSY

SEQ ID NO: 376 - protein, 15 aa, unidentified
  REGION 1..15: note = source = /note="Description of Unknown: APOH49-63 sequence"
YSCKPGYVSRGGMRK

SEQ ID NO: 377 - protein, 15 aa, unidentified
  REGION 1..15: note = source = /note="Description of Unknown: APOH269-283 sequence"
KKATVVYQGERVKIQ

SEQ ID NO: 378 - protein, 15 aa, unidentified
  REGION 1..15: note = source = /note="Description of Unknown: APOH295-309 sequence"
KVSFFCKNKEKKCSY

SEQ ID NO: 379 - protein, 15 aa, unidentified
  REGION 1..15: note = source = /note="Description of Unknown: APOH321-355 sequence"
EVPKCFKEHSSLAFW

SEQ ID NO: 380 - protein, 15 aa, unidentified
  REGION 1..15: note = source = /note="Description of Unknown: APOH322-336 sequence"
VPKCFKEHSSLAFWK

SEQ ID NO: 381 - protein, 15 aa, unidentified
  REGION 1..15: note = source = /note="Description of Unknown: APOH324-338 sequence"
KCFKEHSSLAFWKTD

SEQ ID NO: 382 - protein, 15 aa, unidentified
  REGION 1..15: note = source = /note="Description of Unknown: MPO506-520 sequence"
QPFMFRLDNRYQPME

SEQ ID NO: 383 - protein, 15 aa, unidentified
  REGION 1..15: note = source = /note="Description of Unknown: MPO302-316 sequence"
RIKNQADCIPFFRSC

SEQ ID NO: 384 - protein, 15 aa, unidentified
  REGION 1..15: note = source = /note="Description of Unknown: MPO7-21 sequence"
SSLRCMVDLGPCWAG

SEQ ID NO: 385 - protein, 15 aa, unidentified
  REGION 1..15: note = source = /note="Description of Unknown: MPO689-703 sequence"
QQRQALAQISLPRII

SEQ ID NO: 386 - protein, 15 aa, unidentified
  REGION 1..15: note = source = /note="Description of Unknown: MPO248-262 sequence"
RSLMFMQWGQLLDHD

SEQ ID NO: 387 - protein, 15 aa, unidentified
  REGION 1..15: note = source = /note="Description of Unknown: MPO444-458 sequence"
QEARKIVGAMVQIIT

SEQ ID NO: 388 - protein, 15 aa, unidentified
  REGION 1..15: note = source = /note="Description of Unknown: MPO513-527 sequence"
DNRYQPMEPNPRVPL

SEQ ID NO: 389 - protein, 15 aa, unidentified
  REGION 1..15: note = source = /note="Description of Unknown: MPO97-111 sequence"
ELLSYFKQPVAATRT

SEQ ID NO: 390 - protein, 15 aa, unidentified
  REGION 1..15: note = source = /note="Description of Unknown: MPO616-630 sequence"
QLGTVLRNLKLARKL

SEQ ID NO: 391 - protein, 15 aa, unidentified
  REGION 1..15: note = source = /note="Description of Unknown: MPO462-476 sequence"
YLPLVLGPTAMRKYL

SEQ ID NO: 392 - protein, 15 aa, unidentified
  REGION 1..15: note = source = /note="Description of Unknown: MPO617-631 sequence"
LGTVLRNLKLARKLM

SEQ ID NO: 393 - protein, 15 aa, unidentified
  REGION 1..15: note = source = /note="Description of Unknown: MPO714-728 sequence"
KNNIFMSNSYPRDFV

SEQ ID NO: 394 - protein, 15 aa, unidentified
  REGION 1..15: note = source = /note="Description of Unknown: PRTN344-58 sequence"
SLQMRGNPGSHFCGG

SEQ ID NO: 395 - protein, 15 aa, unidentified
  REGION 1..15: note = source = /note="Description of Unknown: PRTN3234-248 sequence"
TRVALYVDWIRSTLR

SEQ ID NO: 396 - protein, 15 aa, unidentified
  REGION 1..15: note = source = /note="Description of Unknown: PRTN359-73 sequence"
TLIHPSFVLTAAHCL

SEQ ID NO: 397 - protein, 15 aa, unidentified
  REGION 1..15: note = source = /note="Description of Unknown: PRTN3117-131 sequence"
NDVLLIQLSSPANLS

SEQ ID NO: 398 - protein, 15 aa, unidentified
  REGION 1..15: note = source = /note="Description of Unknown: PRTN3164-178 sequence"
DPPAQVLQELNVTVV

SEQ ID NO: 399 - protein, 15 aa, unidentified
  REGION 1..15: note = source = /note="Description of Unknown: PRTN371-85 sequence"
HCLRDIPQRLVNVVL

SEQ ID NO: 400 - protein, 15 aa, unidentified
  REGION 1..15: note = source = /note="Description of Unknown: PRTN3241-255 sequence"
DWIRSTLRRVEAKGR

SEQ ID NO: 401 - protein, 15 aa, unidentified
  REGION 1..15: note = source = /note="Description of Unknown: PRTN359-73 sequence"
TLIHPSFVLTAAHCL

SEQ ID NO: 402 - protein, 15 aa, unidentified
  REGION 1..15: note = source = /note="Description of Unknown: PRTN3183-197 sequence"
RPHNICTFVPRRKAG

SEQ ID NO: 403 - protein, 15 aa, unidentified
  REGION 1..15: note = source = /note="Description of Unknown: PRTN362-76 sequence"
HPSFVLTAAHCLRDI

SEQ ID NO: 404 - protein, 15 aa, unidentified
  REGION 1..15: note = source = /note="Description of Unknown: PRTN3118-132 sequence"
DVLLIQLSSPANLSA

SEQ ID NO: 405 - protein, 15 aa, unidentified
  REGION 1..15: note = source = /note="Description of Unknown: PRTN3239-253 sequence"
YVDWIRSTLRRVEAK

SEQ ID NO: 406 - protein, 15 aa, unidentified
  REGION 1..15: note = source = /note="Description of Unknown: GAD212-226 sequence"
EYVTLKKMREIIGWP

SEQ ID NO: 407 - protein, 15 aa, unidentified
  REGION 1..15: note = source = /note="Description of Unknown: GAD555-569 sequence"
NFFRMVISNPAATHQ

SEQ ID NO: 408 - protein, 15 aa, unidentified
  REGION 1..15: note = source = /note="Description of Unknown: GAD297-311 sequence"
DSVILIKCDERGKMI

SEQ ID NO: 409 - protein, 6 aa, synthetic construct
  REGION 1..6: note = source = /note="Description of Artificial Sequence: Synthetic 6xHis tag"
HHHHHH